European Patent Application EP 4 527 408 A2, published March 26, 2025. Title: CLAUDIN-6 ANTIBODIES AND DRUG CONJUGATES. Applicant: THE REGENTS OF THE UNIVERSITY OF CALIFORNIA. The sequence listing filed with the application follows.

SEQUENCE LISTING (513 sequences)

SEQ ID NO: 1 - protein, 220 aa, Homo sapiens
  REGION 1..220: note = NCBI / NP_067018.2, 2017-06-04
MASAGMQILGVVLTLLGWVNGLVSCALPMWKVTAFIGNSIVVAQVVWEGLWMSCVVQSTGQMQCKVYDSLLALPQDLQAARALCVIALLVALFGLLVYLAGAKCTTCVEEKDSKARLVLTSGIVFVISGVLTLIPVCWTAHAIIRDFYNPLVAEAQKRELGASLYLGWAASGLLLLGGGLLCCTCPSGGSQGPSHYMARYSTSAPAISRGPSEYPTKNYV

SEQ ID NO: 2 - protein, 23 aa, Homo sapiens
WTAHAIIRDFYNPLVAEAQKREL

SEQ ID NO: 3 - protein, 13 aa, Homo sapiens
TAHAIIRDFYNPL

SEQ ID NO: 4 - protein, 10 aa, Homo sapiens
LVAEAQKREL

SEQ ID NO: 5 - protein, 220 aa, Homo sapiens
  REGION 1..220: note = NCBI / NP_001297.1, 2017-07-10
MSMGLEITGTALAVLGWLGTIVCCALPMWRVSAFIGSNIITSQNIWEGLWMNCVVQSTGQMQCKVYDSLLALPQDLQAARALIVVAILLAAFGLLVALVGAQCTNCVQDDTAKAKITIVAGVLFLLAALLTLVPVSWSANTIIRDFYNPVVPEAQKREMGAGLYVGWAAAALQLLGGALLCCSCPPREKKYTATKVVYSAPRSTGPGASLGTGYDRKDYV

SEQ ID NO: 6 - protein, 209 aa, Homo sapiens
  REGION 1..209: note = NCBI / NP_001296.1, 2017-07-10
MASMGLQVMGIALAVLGWLAVMLCCALPMWRVTAFIGSNIVTSQTIWEGLWMNCVVQSTGQMQCKVYDSLLALPQDLQAARALVIISIIVAALGVLLSVVGGKCTNCLEDESAKAKTMIVAGVVFLLAGLMVIVPVSWTAHNIIQDFYNPLVASGQKREMGASLYVGWAASGLLLLGGGLLCCNCPPRTDKPYSAKYSAARSAAASNYV

SEQ ID NO: 7 - protein, 217 aa, Homo sapiens
  REGION 1..217: note = NCBI / NP_066192.1, 2017-04-15
MASTGLELLGMTLAVLGWLGTLVSCALPLWKVTAFIGNSIVVAQVVWEGLWMSCVVQSTGQMQCKVYDSLLALPQDLQAARALCVIALLLALLGLLVAITGAQCTTCVEDEGAKARIVLTAGVILLLAGILVLIPVCWTAHAIIQDFYNPLVAEALKRELGASLYLGWAAAALLMLGGGLLCCTCPPPQVERPRGPRLGYSIPSRSGASGLDKRDYV

SEQ ID NO: 8 - protein, 7 aa, synthetic construct
  REGION 1..7: note = Synthetic peptide
SSVSSTY

SEQ ID NO: 9 - skipped

SEQ ID NO: 10 - protein, 9 aa, synthetic construct
  REGION 1..9: note = Synthetic peptide
HQYHRSPLT

SEQ ID NO: 11 - protein, 8 aa, synthetic construct
  REGION 1..8: note = Synthetic peptide
GYTFTTYT

SEQ ID NO: 12 - protein, 8 aa, synthetic construct
  REGION 1..8: note = Synthetic peptide
INPSSGYT

SEQ ID NO: 13 - protein, 9 aa, synthetic construct
  REGION 1..9: note = Synthetic peptide
ANGDYYVAY

SEQ ID NO: 14 - protein, 6 aa, synthetic construct
  REGION 1..6: note = Synthetic peptide
ENIYSY

SEQ ID NO: 15 - skipped

SEQ ID NO: 16 - protein, 9 aa, synthetic construct
  REGION 1..9: note = Synthetic peptide
QHHYTVPWT

SEQ ID NO: 17 - protein, 8 aa, synthetic construct
  REGION 1..8: note = Synthetic peptide
GFTFSDYW

SEQ ID NO: 18 - protein, 10 aa, synthetic construct
  REGION 1..10: note = Synthetic peptide
IRLKSDNYAT

SEQ ID NO: 19 - protein, 8 aa, synthetic construct
  REGION 1..8: note = Synthetic peptide
NDGPPSGC

SEQ ID NO: 20 - protein, 6 aa, synthetic construct
  REGION 1..6: note = Synthetic peptide
ENIYSY

SEQ ID NO: 21 - skipped

SEQ ID NO: 22 - protein, 9 aa, synthetic construct
  REGION 1..9: note = Synthetic peptide
QHHYTVPWT

SEQ ID NO: 23 - protein, 8 aa, synthetic construct
  REGION 1..8: note = Synthetic peptide
GFTFSNYW

SEQ ID NO: 24 - protein, 10 aa, synthetic construct
  REGION 1..10: note = Synthetic peptide
IRLKSDNYAT

SEQ ID NO: 25 - protein, 8 aa, synthetic construct
  REGION 1..8: note = Synthetic peptide
NDGPPSGC

SEQ ID NO: 26 - protein, 11 aa, synthetic construct
  REGION 1..11: note = Synthetic peptide
QSLVHSDGNTY

SEQ ID NO: 27 - skipped

SEQ ID NO: 28 - protein, 9 aa, synthetic construct
  REGION 1..9: note = Synthetic peptide
SQSTHVPYT

SEQ ID NO: 29 - protein, 8 aa, synthetic construct
  REGION 1..8: note = Synthetic peptide
GYTFTSYT

SEQ ID NO: 30 - protein, 8 aa, synthetic construct
  REGION 1..8: note = Synthetic peptide
INPSSTYT

SEQ ID NO: 31 - protein, 10 aa, synthetic construct
  REGION 1..10: note = Synthetic peptide
SRGELGGFAY

SEQ ID NO: 32 - protein, 11 aa, synthetic construct
  REGION 1..11: note = Synthetic peptide
QSIVHSNGNTY

SEQ ID NO: 33 - skipped

SEQ ID NO: 34 - protein, 9 aa, synthetic construct
  REGION 1..9: note = Synthetic peptide
FQGSHVPFT

SEQ ID NO: 35 - protein, 8 aa, synthetic construct
  REGION 1..8: note = Synthetic peptide
GYIFTHYI

SEQ ID NO: 36 - protein, 8 aa, synthetic construct
  REGION 1..8: note = Synthetic peptide
INPYNDGT

SEQ ID NO: 37 - protein, 13 aa, synthetic construct
  REGION 1..13: note = Synthetic peptide
ARYYGYPYYSMDY

SEQ ID NO: 38 - protein, 12 aa, synthetic construct
  REGION 1..12: note = Synthetic peptide
QSLLNSRTRKNY

SEQ ID NO: 39 - skipped

SEQ ID NO: 40 - protein, 8 aa, synthetic construct
  REGION 1..8: note = Synthetic peptide
KQSYYLYT

SEQ ID NO: 41 - protein, 9 aa, synthetic construct
  REGION 1..9: note = Synthetic peptide
GYSITSGYY

SEQ ID NO: 42 - protein, 7 aa, synthetic construct
  REGION 1..7: note = Synthetic peptide
ISYDGGI

SEQ ID NO: 43 - protein, 10 aa, synthetic construct
  REGION 1..10: note = Synthetic peptide
ARFGKGAMDY

SEQ ID NO: 44 - protein, 7 aa, synthetic construct
  REGION 1..7: note = Synthetic peptide
SSVSSSY

SEQ ID NO: 45 - skipped

SEQ ID NO: 46 - protein, 9 aa, synthetic construct
  REGION 1..9: note = Synthetic peptide
HQYHRSPPT

SEQ ID NO: 47 - protein, 8 aa, synthetic construct
  REGION 1..8: note = Synthetic peptide
GYSFTGYT

SEQ ID NO: 48 - protein, 8 aa, synthetic construct
  REGION 1..8: note = Synthetic peptide
INPYNGGT

SEQ ID NO: 49 - protein, 12 aa, synthetic construct
  REGION 1..12: note = Synthetic peptide
ARGVYDYDGFTY

SEQ ID NO: 50 - protein, 11 aa, synthetic construct
  REGION 1..11: note = Synthetic peptide
QSLVHSDGNTY

SEQ ID NO: 51 - skipped

SEQ ID NO: 52 - protein, 9 aa, synthetic construct
  REGION 1..9: note = Synthetic peptide
SQSTHVPYT

SEQ ID NO: 53 - protein, 8 aa, synthetic construct
  REGION 1..8: note = Synthetic peptide
GYTFTTYT

SEQ ID NO: 54 - protein, 8 aa, synthetic construct
  REGION 1..8: note = Synthetic peptide
INPRSGYS

SEQ ID NO: 55 - protein, 10 aa, synthetic construct
  REGION 1..10: note = Synthetic peptide
SRGELGGFAY

SEQ ID NO: 56 - protein, 6 aa, synthetic construct
  REGION 1..6: note = Synthetic peptide
QTIGTW

SEQ ID NO: 57 - skipped

SEQ ID NO: 58 - protein, 9 aa, synthetic construct
  REGION 1..9: note = Synthetic peptide
QQLYSIPRT

SEQ ID NO: 59 - protein, 8 aa, synthetic construct
  REGION 1..8: note = Synthetic peptide
GYRFTDYN

SEQ ID NO: 60 - protein, 8 aa, synthetic construct
  REGION 1..8: note = Synthetic peptide
INPNNGGT

SEQ ID NO: 61 - protein, 10 aa, synthetic construct
  REGION 1..10: note = Synthetic peptide
ARDYLYFFDC

SEQ ID NO: 62 - protein, 11 aa, synthetic construct
  REGION 1..11: note = Synthetic peptide
QSLVHSNGNTY

SEQ ID NO: 63 - skipped

SEQ ID NO: 64 - protein, 9 aa, synthetic construct
  REGION 1..9: note = Synthetic peptide
SQITHVPYT

SEQ ID NO: 65 - protein, 8 aa, synthetic construct
  REGION 1..8: note = Synthetic peptide
GYTFTDYS

SEQ ID NO: 66 - protein, 8 aa, synthetic construct
  REGION 1..8: note = Synthetic peptide
ISTETGEP

SEQ ID NO: 67 - protein, 10 aa, synthetic construct
  REGION 1..10: note = Synthetic peptide
TRGLWSSFAY

SEQ ID NO: 68 - protein, 10 aa, synthetic construct
  REGION 1..10: note = Synthetic peptide
KSVSTSGYSY

SEQ ID NO: 69 - skipped

SEQ ID NO: 70 - protein, 9 aa, synthetic construct
  REGION 1..9: note = Synthetic peptide
QHSRELPLT

SEQ ID NO: 71 - protein, 8 aa, synthetic construct
  REGION 1..8: note = Synthetic peptide
GFTFSSFG

SEQ ID NO: 72 - protein, 8 aa, synthetic construct
  REGION 1..8: note = Synthetic peptide
ISSDSRTI

SEQ ID NO: 73 - protein, 11 aa, synthetic construct
  REGION 1..11: note = Synthetic peptide
ARDYGRTYEAY

SEQ ID NO: 74 - protein, 6 aa, synthetic construct
  REGION 1..6: note = Synthetic peptide
QDIGGN

SEQ ID NO: 75 - skipped

SEQ ID NO: 76 - protein, 9 aa, synthetic construct
  REGION 1..9: note = Synthetic peptide
LQRNAYPLT

SEQ ID NO: 77 - protein, 8 aa, synthetic construct
  REGION 1..8: note = Synthetic peptide
GFTFSSYA

SEQ ID NO: 78 - protein, 7 aa, synthetic construct
  REGION 1..7: note = Synthetic peptide
IRSGGTT

SEQ ID NO: 79 - protein, 12 aa, synthetic construct
  REGION 1..12: note = Synthetic peptide
AKVGGNPYPMDY

SEQ ID NO: 80 - protein, 7 aa, synthetic construct
  REGION 1..7: note = Synthetic peptide
SSISSNY

SEQ ID NO: 81 - skipped

SEQ ID NO: 82 - protein, 9 aa, synthetic construct
  REGION 1..9: note = Synthetic peptide
QQGSSIPLT

SEQ ID NO: 83 - protein, 8 aa, synthetic construct
  REGION 1..8: note = Synthetic peptide
GYAFSNYL

SEQ ID NO: 84 - protein, 8 aa, synthetic construct
  REGION 1..8: note = Synthetic peptide
INPGSGGT

SEQ ID NO: 85 - protein, 15 aa, synthetic construct
  REGION 1..15: note = Synthetic peptide
ARSYFGRSYPYTMDY

SEQ ID NO: 86 - protein, 10 aa, synthetic construct
  REGION 1..10: note = Synthetic peptide
QSVDYDGDNY

SEQ ID NO: 87 - skipped

SEQ ID NO: 88 - protein, 9 aa, synthetic construct
  REGION 1..9: note = Synthetic peptide
QQSNEDPFT

SEQ ID NO: 89 - protein, 8 aa, synthetic construct
  REGION 1..8: note = Synthetic peptide
GYTFTDYA

SEQ ID NO: 90 - protein, 8 aa, synthetic construct
  REGION 1..8: note = Synthetic peptide
ISTYSGNT

SEQ ID NO: 91 - protein, 13 aa, synthetic construct
  REGION 1..13: note = Synthetic peptide
ARRGDYSLYAMDY

SEQ ID NO: 92 - protein, 12 aa, synthetic construct
  REGION 1..12: note = Synthetic peptide
QSVLFSSNQKNY

SEQ ID NO: 93 - skipped

SEQ ID NO: 94 - protein, 8 aa, synthetic construct
  REGION 1..8: note = Synthetic peptide
HQYLSSRT

SEQ ID NO: 95 - protein, 8 aa, synthetic construct
  REGION 1..8: note = Synthetic peptide
GFTFSSFG

SEQ ID NO: 96 - protein, 8 aa, synthetic construct
  REGION 1..8: note = Synthetic peptide
ISSDSRTI

SEQ ID NO: 97 - protein, 11 aa, synthetic construct
  REGION 1..11: note = Synthetic peptide
ARDYGRTYEAY

SEQ ID NO: 98 - protein, 10 aa, synthetic construct
  REGION 1..10: note = Synthetic peptide
ESVDNYGISF

SEQ ID NO: 99 - skipped

SEQ ID NO: 100 - protein, 9 aa, synthetic construct
  REGION 1..9: note = Synthetic peptide
QQSKEVPLT

SEQ ID NO: 101 - protein, 8 aa, synthetic construct
  REGION 1..8: note = Synthetic peptide
GFPFSSSA

SEQ ID NO: 102 - protein, 7 aa, synthetic construct
  REGION 1..7: note = Synthetic peptide
INSDGNT

SEQ ID NO: 103 - protein, 13 aa, synthetic construct
  REGION 1..13: note = Synthetic peptide
TRNGDYRYDEFAY

SEQ ID NO: 104 - protein, 7 aa, synthetic construct
  REGION 1..7: note = Synthetic peptide
SSVSSSY

SEQ ID NO: 105 - skipped

SEQ ID NO: 106 - protein, 9 aa, synthetic construct
  REGION 1..9: note = Synthetic peptide
HQYHRSPPT

SEQ ID NO: 107 - protein, 8 aa, synthetic construct
  REGION 1..8: note = Synthetic peptide
GYTFTGYW

SEQ ID NO: 108 - protein, 8 aa, synthetic construct
  REGION 1..8: note = Synthetic peptide
INPSTGYT

SEQ ID NO: 109 - protein, 12 aa, synthetic construct
  REGION 1..12: note = Synthetic peptide
AREGITTVLVDY

SEQ ID NO: 110 - protein, 12 aa, synthetic construct
  REGION 1..12: note = Synthetic peptide
QSVLFSSNQKNY

SEQ ID NO: 111 - skipped

SEQ ID NO: 112 - protein, 8 aa, synthetic construct
  REGION 1..8: note = Synthetic peptide
HQYLSSRT

SEQ ID NO: 113 - protein, 8 aa, synthetic construct
  REGION 1..8: note = Synthetic peptide
GYSFTGYN

SEQ ID NO: 114 - protein, 8 aa, synthetic construct
  REGION 1..8: note = Synthetic peptide
IDPYYGGS

SEQ ID NO: 115 - protein, 14 aa, synthetic construct
  REGION 1..14: note = Synthetic peptide
ARERSGYVFSAMDY

SEQ ID NO: 116 - protein, 12 aa, synthetic construct
  REGION 1..12: note = Synthetic peptide
QSVLFSSNQKNY

SEQ ID NO: 117 - skipped

SEQ ID NO: 118 - protein, 8 aa, synthetic construct
  REGION 1..8: note = Synthetic peptide
HQYLSSRT

SEQ ID NO: 119 - protein, 8 aa, synthetic construct
  REGION 1..8: note = Synthetic peptide
GYSFTGYT

SEQ ID NO: 120 - protein, 8 aa, synthetic construct
  REGION 1..8: note = Synthetic peptide
INPYNGVT

SEQ ID NO: 121 - protein, 16 aa, synthetic construct
  REGION 1..16: note = Synthetic peptide
TRDPLYYGYRDSTMDY

SEQ ID NO: 122 - protein, 11 aa, synthetic construct
  REGION 1..11: note = Synthetic peptide
QSLVHSDGNTY

SEQ ID NO: 123 - skipped

SEQ ID NO: 124 - protein, 9 aa, synthetic construct
  REGION 1..9: note = Synthetic peptide
SQSTHVPYT

SEQ ID NO: 125 - protein, 8 aa, synthetic construct
  REGION 1..8: note = Synthetic peptide
GYTFTSYT

SEQ ID NO: 126 - protein, 8 aa, synthetic construct
  REGION 1..8: note = Synthetic peptide
INPSSTYT

SEQ ID NO: 127 - protein, 10 aa, synthetic construct
  REGION 1..10: note = Synthetic peptide
SRGELGGFAY

SEQ ID NO: 128 - protein, 6 aa, synthetic construct
  REGION 1..6: note = Synthetic peptide
QGIRGN

SEQ ID NO: 129 - skipped

SEQ ID NO: 130 - protein, 9 aa, synthetic construct
  REGION 1..9: note = Synthetic peptide
LQRNAYPLT

SEQ ID NO: 131 - protein, 8 aa, synthetic construct
  REGION 1..8: note = Synthetic peptide
GFTFSSFA

SEQ ID NO: 132 - protein, 7 aa, synthetic construct
  REGION 1..7: note = Synthetic peptide
IRSGGIT

SEQ ID NO: 133 - protein, 13 aa, synthetic construct
  REGION 1..13: note = Synthetic peptide
ARVSTATYYGMDY

SEQ ID NO: 134 - protein, 108 aa, synthetic construct
  REGION 1..108: note = Synthetic peptide
QIVLTQSPAIMSASLGERVTMTCTASSSVSSTYFHWYQQKPGSSPKLWIYSTSNLASGVPRRFSGSASGTSYSLTISSMEAEDAATYYCHQYHRSPLTFGAGTKLELK

SEQ ID NO: 135 - protein, 116 aa, synthetic construct
  REGION 1..116: note = Synthetic peptide
QVQLQQSAAELARPGASVKMSCKASGYTFTTYTMHWVKQRPGQGLEWIGFINPSSGYTDYNQKFKDRTTLTADKSSSTVYMQLSSLTSEDSAVYYCANGDYYVAYWGQGTLVTVSA

SEQ ID NO: 136 - protein, 107 aa, synthetic construct
  REGION 1..107: note = Synthetic peptide
DIQMTQSPASLSASVGETVTITCRISENIYSYLAWYQQKQGKSPQLLVYNAKILVEGVPSRFSGSGSGTQFSLKINSLQPEDFGNYYCQHHYTVPWTFGGGTKLEIK

SEQ ID NO: 137 - protein, 117 aa, synthetic construct
  REGION 1..117: note = Synthetic peptide
EVKLEESGGGLVQPGGSMKLSCVASGFTFSDYWMNWVRQSPEKGLEWVAQIRLKSDNYATHYAESVKGRFTISRDDSKRSVYLQMNNLRAEDTGTYYCNDGPPSGCWGQGTTLIVSS

SEQ ID NO: 138 - protein, 107 aa, synthetic construct; identical to SEQ ID NO: 136
  REGION 1..107: note = Synthetic peptide

SEQ ID NO: 139 - protein, 117 aa, synthetic construct
  REGION 1..117: note = Synthetic peptide
EVKLEESGGGLVQPGGSMKLSCVASGFTFSNYWMNWVRQSPEKGLEWVAQIRLKSDNYATHYAESVKGRFTISRDDSKRSVYLQMNNLRAEDTGTYYCNDGPPSGCWGQGTTLIVSS

SEQ ID NO: 140 - protein, 112 aa, synthetic construct
  REGION 1..112: note = Synthetic peptide
DVVMTQTPLSLPVSLGDQASISCRSSQSLVHSDGNTYLNWYLQKPGQSPKLLIYKVSNRFSGVPDRFSGSGSGTDFTLKIRRVEAEDLGVYFCSQSTHVPYTFGGGTKLEIK

SEQ ID NO: 141 - protein, 117 aa, synthetic construct
  REGION 1..117: note = Synthetic peptide
QVQLQQSGAELARPGASVKMSCKASGYTFTSYTMHWIKQRPGQGQEWIGYINPSSTYTHYIKKFKDKATLTADKSSSTAYMQLRSLTSEDSAVYYCSRGELGGFAYWGQGTLVTVSA

SEQ ID NO: 142 - protein, 112 aa, synthetic construct
  REGION 1..112: note = Synthetic peptide
DVLMTQTPLSLPVSLGDQPSISCRSSQSIVHSNGNTYLDWYLQKPGQSPKLLIYKVSNRFSGVPDRFSGSGSGTDFTLKISRVEAEDLGVYYCFQGSHVPFTFGSGTRLEIK

SEQ ID NO: 143 - protein, 120 aa, synthetic construct
  REGION 1..120: note = Synthetic peptide
EVQLQQSGPELVKPGASVKMSCKASGYIFTHYIMHWVKQKPGQGLEWIGCINPYNDGTKYNEKFKGKATLTSDKSSSTAYMELSSLTSEDSAVYYCARYYGYPYYSMDYWGQGTSVTVSS

SEQ ID NO: 144 - protein, 112 aa, synthetic construct
  REGION 1..112: note = Synthetic peptide
AIVMFQSPSSLVVSAGEKVTMSCKSSQSLLNSRTRKNYLAWYQQKPGQSPKLLIYWASTRESGVPDRFTGSGSGTDFTLTISSVQAEDLAVYYCKQSYYLYTFGGGTKLEIK

SEQ ID NO: 145 - protein, 117 aa, synthetic construct
  REGION 1..117: note = Synthetic peptide
DVQLQESGPGLVKSSQSLSLTCSVTGYSITSGYYWKWIRQFPGNKLEWMGYISYDGGINYNPSLKNRISITRDTSKNQFFLKLNSVTTEDTAKYYCARFGKGAMDYWGQGTSVTVSS

SEQ ID NO: 146 - protein, 108 aa, synthetic construct
  REGION 1..108: note = Synthetic peptide
QIVLTQSPAIMSASLGDRVTMTCTASSSVSSSYLHWYQQKPGSSPKLWIYSTSNLASGVPARFSGSGSGTSYSLTISSMEAEDAATYYCHQYHRSPPTFGSGTKLEIK

SEQ ID NO: 147 - protein, 119 aa, synthetic construct
  REGION 1..119: note = Synthetic peptide
EVQLQQSGPELVKPGASMKISCKASGYSFTGYTMNWVKQSHGKNLEWIGLINPYNGGTNYNQKFKGKATLTVDKSSSTAYMELLSLTSEDSAVYYCARGVYDYDGFTYWGQGTLVTVSA

SEQ ID NO: 148 - protein, 112 aa, synthetic construct
  REGION 1..112: note = Synthetic peptide
DVVMTQTPLSLPVSLGDQASISCRSSQSLVHSDGNTYLYWYLQKPGQSPKLLIYKVSNRFSGVPDRFSGSGSGTDFTLKISRVEAEDLGVYFCSQSTHVPYTFGGGTKLEIK

SEQ ID NO: 149 - protein, 117 aa, synthetic construct
  REGION 1..117: note = Synthetic peptide
QVQLQQSGAELARPGASVKMSCKASGYTFTTYTMHWLKQRPGQGLEWIGYINPRSGYSNYNQKFKDKATLTADKSSNTAYMQLNTLTSEDSKVYYCSRGELGGFAYWGQGTLVTVSA

SEQ ID NO: 150 - protein, 107 aa, synthetic construct
  REGION 1..107: note = Synthetic peptide
DIQMTQSPASQSASLGESVTITCLASQTIGTWLAWYQQKPGKSPQLLIYAAASLADGVPSRFSGSGSGTRFSFKISSLQAEDFVSYYCQQLYSIPRTFGGGTKLEIK

SEQ ID NO: 151 - protein, 117 aa, synthetic construct
  REGION 1..117: note = Synthetic peptide
EVQLQQSGPELVKPGASVKMSCKASGYRFTDYNMHWVKQSHGKSLEWIGYINPNNGGTNYNQNFKGKATLTVNKSSSTAYMELRSLTSEDSAAYYCARDYLYFFDCWGQGTTLTVSS

SEQ ID NO: 152 - protein, 112 aa, synthetic construct
  REGION 1..112: note = Synthetic peptide
DVVMTQTPLSLPVSLGDQASISCRASQSLVHSNGNTYLHWFLQKPGQSPKLLIYKVSNRFSGVPDRFSGSGSRTDFTLKISRVEAEDLGVYFCSQITHVPYTFGGGTKLEIK

SEQ ID NO: 153 - protein, 117 aa, synthetic construct
  REGION 1..117: note = Synthetic peptide
QIQLVQSGPALKKPGETVKISCKASGYTFTDYSMHWIKQAPGKGLKWMGWISTETGEPTYADGFKGRFDFSLETSADTAYLSINNLTNEDTATYFCTRGLWSSFAYWGQGTLVTVSA

SEQ ID NO: 154 - protein, 111 aa, synthetic construct
  REGION 1..111: note = Synthetic peptide
DIVLTQSPASLAVSLGQRATISCRASKSVSTSGYSYIHWYQQKPGQPPKLLIYLASNLESGVPARFSGSGSGTDFTLNIHPVEEEDAATYYCQHSRELPLTFGAGTKLELK

SEQ ID NO: 155 - protein, 118 aa, synthetic construct
  REGION 1..118: note = Synthetic peptide
DVQLVESGGGLVQPRGSRKLSCAASGFTFSSFGMHWVRQAPEKGLEWVAYISSDSRTIYYADTVKGRFTISRDNPTNTLFLQMTSLRSEDTAMYYCARDYGRTYEAYWGQGTLVTVSA

SEQ ID NO: 156 - protein, 107 aa, synthetic construct
  REGION 1..107: note = Synthetic peptide
DIQMIQSPSSMFASLGDRVSLSCRASQDIGGNLDWYQQKPGGTIKLLIYSTSNLNSGVPSRFSGSGSGSDYSLTITSLESEDFADYYCLQRNAYPLTFGAGTKLELK

SEQ ID NO: 157 - protein, 118 aa, synthetic construct
  REGION 1..118: note = Synthetic peptide
EVKLMESGGDLVKPGGSLKLSCAASGFTFSSYAMSWVRQTPEKRLEWVASIRSGGTTYYPDSVKGRFTISRDNARNILYLRMSSLRSEDTAIYYCAKVGGNPYPMDYWGQGTSVTVSS

SEQ ID NO: 158 - protein, 108 aa, synthetic construct
  REGION 1..108: note = Synthetic peptide
EIVLTQSPTTMAASPGEKITITCSASSSISSNYLHWYQQKPGFSPKLLIYRTSNLASGVPARFSGSGSGTSYSLTIGTMEAEDVATYYCQQGSSIPLTFGAGTKLELK

SEQ ID NO: 159 - protein, 122 aa, synthetic construct
  REGION 1..122: note = Synthetic peptide
QVQLQQSGAELVRPGTSVKVSCKASGYAFSNYLIEWVKQRPGQGLEWIGVINPGSGGTNYNEKFKGKATMTADKSSSTAYMHLSNLTSEDSVVYFCARSYFGRSYPYTMDYWGQGTSVTVSS

SEQ ID NO: 160 - protein, 111 aa, synthetic construct
  REGION 1..111: note = Synthetic peptide
DIVLTQSPASLAVSLGQRATISCKASQSVDYDGDNYVNWYQQKVGQPPKLLISAASNLESGIPARFSGSGSGTDFTLNIHPVEEEDAATYYCQQSNEDPFTFGSGTKLEIK

SEQ ID NO: 161 - protein, 120 aa, synthetic construct
  REGION 1..120: note = Synthetic peptide
QVQLQQSGPELVRPGVSVKISCKGSGYTFTDYAMHWVKQSHAKSLEWIGVISTYSGNTNYNQKFQDKATMTVDKSSSTAYMALARLTSDDSAIYYCARRGDYSLYAMDYWGQGTSVTVSS

SEQ ID NO: 162 - protein, 112 aa, synthetic construct
  REGION 1..112: note = Synthetic peptide
NIMMTQSPSSLAVSAGEKVTMSCKSSQSVLFSSNQKNYLAWYQQKPGQSPRLLIYWASTRESGVPDRFTGSGSGTDFTLTISNVQAEDLAVYYCHQYLSSRTFGAGTKLELK

SEQ ID NO: 163 - protein, 118 aa, synthetic construct; identical to SEQ ID NO: 155
  REGION 1..118: note = Synthetic peptide

SEQ ID NO: 164 - protein, 111 aa, synthetic construct
  REGION 1..111: note = Synthetic peptide
DIVLTQSPASLALSLGQRATISCRASESVDNYGISFMNWFQQKPGQPPKLLIYAASNQGSGVPARFSGSGSGTDFSLNIHPMEEDDTAMYFCQQSKEVPLTFGAGTKLELK

SEQ ID NO: 165 - protein, 119 aa, synthetic construct
  REGION 1..119: note = Synthetic peptide
EVRLVESGGGLMQPGGSLKLPCAASGFPFSSSAMSWVRQTPEKRLEWVASINSDGNTYYPDSVKGRFTISRDSARNILYLQMSSLRSEDTAMYYCTRNGDYRYDEFAYWGQGTLVTVSA

SEQ ID NO: 166 - protein, 108 aa, synthetic construct
  REGION 1..108: note = Synthetic peptide
QIVLTQSPAIMSASLGERVTMTCTASSSVSSSYLHWYQQKPGSSPKLWIYSTSNLASGVPARFSGSGSGTSYSLTISSMEAEDAATYYCHQYHRSPPTFGAGTKLELK

SEQ ID NO: 167 - protein, 119 aa, synthetic construct
  REGION 1..119: note = Synthetic peptide
QVQLQQSGAELAKPGASVKMSCKASGYTFTGYWMHWVKQRPGQGLEWLGYINPSTGYTESNQKFKDKATLTADKSSTTAYMQLRSLTPEDSAVYYCAREGITTVLVDYWGQGTTLTVSS

SEQ ID NO: 168 - protein, 112 aa, synthetic construct; identical to SEQ ID NO: 162
  REGION 1..112: note = Synthetic peptide

SEQ ID NO: 169 - protein, 121 aa, synthetic construct
  REGION 1..121: note = Synthetic peptide
QVQLKQSGPELEKPGASVKISCKASGYSFTGYNMNWVKQSNGKSLEWIGNIDPYYGGSTYNQKFTGKATLTVDKSSSTAYMQLKSLTSEDSAVYYCARERSGYVFSAMDYWGQGTSVTVSS

SEQ ID NO: 170 - protein, 112 aa, synthetic construct; identical to SEQ ID NO: 162
  REGION 1..112: note = Synthetic peptide

SEQ ID NO: 171 - protein, 123 aa, synthetic construct
  REGION 1..123: note = Synthetic peptide
EVQLQQSGPELVKPGGSMKISCKASGYSFTGYTMNWVKRSHGKNLEWIGLINPYNGVTTYNQNFKGKATLAVDKSSSTAYMELLGLTSEDSAVYYCTRDPLYYGYRDSTMDYWGQGTSVTVSS

SEQ ID NO: 172 - protein, 112 aa, synthetic construct; identical to SEQ ID NO: 140
  REGION 1..112: note = Synthetic peptide

SEQ ID NO: 173 - protein, 117 aa, synthetic construct
  REGION 1..117: note = Synthetic peptide
EVQLQQSGAELARPGASVKMSCKASGYTFTSYTMHWIKQRPGQGQEWIGYINPSSTYTHYIKKFKDKATLTADKSSSTAYMQLRSLTSEDSAVYYCSRGELGGFAYWGQGTLVTVSA

SEQ ID NO: 174 - protein, 107 aa, synthetic construct
  REGION 1..107: note = Synthetic peptide
DIQMIQSPSSMFASLGDRVSLSCRASQGIRGNLDWYQQKPGGTIKLLIYSTSILNSGVPSRFSGSGSGSDYSLTITSLESEDFADYYCLQRNAYPLTFGSGTKLELK

SEQ ID NO: 175 - protein, 119 aa, synthetic construct
  REGION 1..119: note = Synthetic peptide
EVKLVESGGGLMKPGGSLKLSCAASGFTFSSFALSWVRQTPEKRLEWVASIRSGGITYHADSVKGRFTISRDNAGNILYLQMNSLRSEDTAMYFCARVSTATYYGMDYWGQGTSVTVSS

SEQ ID NO: 176 - protein, 219 aa, Mus musculus
  REGION 1..219: note = NCBI / NP_061247.1, 2017-08-07
MASTGLQILGIVLTLLGWVNALVSCALPMWKVTAFIGNSIVVAQMVWEGLWMSCVVQSTGQMQCKVYDSLLALPQDLQAARALCVVTLLIVLLGLLVYLAGAKCTTCVEDRNSKSRLVLISGIIFVISGVLTLIPVCWTAHSIIQDFYNPLVADAQKRELGASLYLGWAASGLLLLGGGLLCCACSSGGTQGPRHYMACYSTSVPHSRGPSEYPTKNYV

SEQ ID NO: 177 - protein, 80 aa, synthetic construct
  REGION 1..80: note = Synthetic peptide
MASAGMQILGVVLTLLGWVNGLVSCALPMWKVTAFIGNSIVVAQVVWEGLWMSCVVQSTGQMQCKVYDSLLALPQDLQAA

SEQ ID NO: 178 - protein, 220 aa, synthetic construct
  REGION 1..220: note = Synthetic peptide
MASAGMQILGVVLTLLGWVNGLVSCALPMWKVTAFIGNSIVVAQVVWEGLWMSCVVQSTGQMQCKVYDSLLALPQDLQAARALCVIALLVALFGLLVYLAGAKCTTCVEEKDSKARLVLTSGIVFVISGVLTLIPVCWTAHAVIRDFYNPLVAEAQKRELGASLYLGWAASGLLLLGGGLLCCTCPSGGSQGPSHYMARYSTSAPAISRGPSEYPTKNYV

SEQ ID NO: 179 - protein, 322 aa, synthetic construct
  REGION 1..322: note = Synthetic peptide
CAGATCGTGCTGACTCAGAGTCCTTCAATTATGTCCGTGAGCCCAGGCGAGAAGGTCACCATCACATGCAGTGCCTCCAGCTCTGTCTCATACATGCACTGGTTCCAGCAGAAGCCAGGGACCAGTCCCAAGCTGTGCATCTACTCTACATCGAACCTGGCCTCCGGAGTGCCCGCAAGGTTTAGCGGTCGGGGCTCTGGAACTTCATACTCCCTGACCATCTCGCGGGTGGCCGCTGAGGATGCAGCAACATACTATTGCCAGCAGAGGTCCAATTATCCCCCTTGGACATTCGGCGGAGGTACCAAACTCGAGATTAAGC

SEQ ID NO: 180 - protein, 351 aa, synthetic construct
  REGION 1..351: note = Synthetic peptide
GAAGTCCAGCTGCAGCAGTCTGGCCCTGAACTGGTGAAGCCTGGCGCCAGCATGAAGATCTCCTGCAAGGCCAGCGGCTACTCCTTCACCGGCTATACAATGAACTGGGTGAAGCAGTCCCACGGCAAGAATCTGGAGTGGATCGGCCTGATCAACCCATACAATGGCGGCACCATCTACAACCAGAAGTTTAAGGGCAAGGCCACCCTGACAGTGGACAAGAGCTCCTCTACCGCCTACATGGAGCTGCTGTCTCTGACAAGCGAGGACTCCGCCGTGTACTATTGCGCCCGGGACTACGGCTTCGTGCTGGACTATTGGGGCCAGGGCACCACACTGACAGTGAGCTCC

SEQ ID NO: 181 - protein, 107 aa, synthetic construct
  REGION 1..107: note = Synthetic peptide
QIVLTQSPSIMSVSPGEKVTITCSASSSVSYMHWFQQKPGTSPKLCIYSTSNLASGVPARFSGRGSGTSYSLTISRVAAEDAATYYCQQRSNYPPWTFGGGTKLEIK

SEQ ID NO: 182 - protein, 117 aa, synthetic construct
  REGION 1..117: note = Synthetic peptide
EVQLQQSGPELVKPGASMKISCKASGYSFTGYTMNWVKQSHGKNLEWIGLINPYNGGTIYNQKFKGKATLTVDKSSSTAYMELLSLTSEDSAVYYCARDYGFVLDYWGQGTTLTVSS

SEQ ID NO: 183 - DNA, 324 bp, synthetic construct
  misc_feature 1..324: note = Synthetic polynucleotide
  source 1..324: mol_type = other DNA
gaaattgtgctcacccagtctccagcactcatggctgcatctccaggggagaaggtcaccatcacctgcagtgtcagctcaagtataagttccagcaacttgcactggtaccagcagaagtcaggaacctcccccaaactctggatttatggcacatccaacctggcttctggagtccctgttcgcttcagtggcagtggatctgggacctcttattctctcacaatcagcaacatggaggctgaagatgctgccacttattactgtcaacagtggagtagttacccacacacgttcggaggggggaccaagctggaaataaaa

SEQ ID NO: 184 - DNA, 378 bp, synthetic construct
  misc_feature 1..378: note = Synthetic polynucleotide
  source 1..378: mol_type = other DNA
caggtccaaatgcagcagtctggagctgagctggtaaggcctgggacttcagtgaaggtgtcctgcaaggcttctggatacgccttcactaattacttgatagagtgggtaaagcagaggcctggacagggccttgagtggattggactgattaatcctggaagtggtggtactaattacaatgagaagttcaagggcaaggcaacactgactgcagacaaatcctccaccactgcctacatgcagctcagcagcctgacatctgatgactctgcggtttatttctgtgcaagacggtcccctctagggagttggatctactatgcttacgacggtgttgcttactggggccaagggactctggtcactgtctctgca

SEQ ID NO: 185 - protein, 108 aa, synthetic construct
  REGION 1..108: note = Synthetic peptide
EIVLTQSPALMAASPGEKVTITCSVSSSISSSNLHWYQQKSGTSPKLWIYGTSNLASGVPVRFSGSGSGTSYSLTISNMEAEDAATYYCQQWSSYPHTFGGGTKLEIK

SEQ ID NO: 186 - protein, 126 aa, synthetic construct
  REGION 1..126: note = Synthetic peptide
QVQMQQSGAELVRPGTSVKVSCKASGYAFTNYLIEWVKQRPGQGLEWIGLINPGSGGTNYNEKFKGKATLTADKSSTTAYMQLSSLTSDDSAVYFCARRSPLGSWIYYAYDGVAYWGQGTLVTVSA

SEQ ID NO: 187 - DNA, 645 bp, Mus musculus
  source 1..645: mol_type = genomic DNA
gatattgtgctaactcagtctccagccaccctgtctgtgactccaggaaatagcgtcagtctttcctgcagggccagccaaagtattggcggtaacctacactggtatcaacaaaaatcacatgagtctccaaggcttctcatcaagtatgcttcccagtccatctctgggatcccctccaggttcagtggcagtggatcagggacagatttcactctcagtatcaacagtgtggagactgaagattttggaatgtatttctgtcaacagagtaacagctggccttacacgttcggaggggggaccaagctggaaataaaacgggcagatgctgcaccaactgtatccatcttcccaccatccagtgagcagttaacatctggaggtgcctcagtcgtgtgcttcttgaacaacttctaccccaaagacatcaatgtcaagtggaagattgatggcagtgaacgacaaaatggcgtcctgaacagttggactgatcaggacagcaaagacagcacctacagcatgagcagcaccctcacgttgaccaaggacgagtatgaacgacataacagctatacctgtgaggccactcacaagacatcaacttcacccattgtcaagagcttcaacaggaatgagtgttag

SEQ ID NO: 188 - DNA, 1335 bp, Mus musculus
  source 1..1335: mol_type = genomic DNA
gacgtgcagcttcaggagtcaggacctagcctcgtgaaaccttctcagactctgtccctcacctgttctgtcactggcgactccatcaccagtgattactggagctggatccggaaattcccagggaatagacttgagtacatggggtacgtaagctacagtggtagcacttactacaatccatctctcaaaagtcgaatctccatcacccgagacacatccaagaaccagtactacctggatttgaattctgtgactactgaggacacagccacatattactgtgcaaactgggacggtgattactggggccaagggactctggtcactgtctcttcagcagctaaaacaacagccccatcggtctatccactggcccctgtgtgtggagatacaactggctcctcggtgactctaggatgcctggtcaagggttatttccctgagccagtgaccttgacctggaactctggatccctgtccagtggtgtgcacaccttcccagctgtcctgcagtctgacctctacaccctcagcagctcagtgactgtaacctcgagcacctggcccagccagtccatcacctgcaatgtggcccacccggcaagcagcaccaaggtggacaagaaaattgagcccagagggcccacaatcaagccctgtcctccatgcaaatgcccagcacctaacctcttgggtggaccatccgtcttcatcttccctccaaagatcaaggatgtactcatgatctccctgagccccatagtcacatgtgtggtggtggatgtgagcgaggatgacccagatgtccagatcagctggtttgtgaacaacgtggaagtacacacagctcagacacaaacccatagagaggattacaacagtactctccgggtggtcagtgccctccccatccagcaccaggactggatgagtggcaaggagttcaaatgcaaggtcaacaacaaagacctcccagcgcccatcgagagaaccatctcaaaacccaaagggtcagtaagagctccacaggtatatgtcttgcctccaccagaagaagagatgactaagaaacaggtcactctgacctgcatggtcacagacttcatgcctgaagacatttacgtggagtggaccaacaacgggaaaacagagctaaactacaagaacactgaaccagtcctggactctgatggttcttacttcatgtacagcaagctgagagtggaaaagaagaactgggtggaaagaaatagctactcctgttcagtggtccacgagggtctgcacaatcaccacacgactaagagcttctcccggactccgggtaaatga

SEQ ID NO: 189 - DNA, 8806 bp, synthetic construct
  misc_feature 1..8806: note = Synthetic peptide
  source 1..8806: mol_type = other DNA
aatgtagtcttatgcaatactcttgtagtcttgcaacatggtaacgatgagttagcaacatgccttacaaggagagaaaaagcaccgtgcatgccgattggtggaagtaaggtggtacgatcgtgccttattaggaaggcaacagacgggtctgacatggattggacgaaccactgaattgccgcattgcagagatattgtatttaagtgcctagctcgatacataaacgggtctctctggttagaccagatctgagcctgggagctctctggctaactagggaacccactgcttaagcctcaataaagcttgccttgagtgcttcaagtagtgtgtgcccgtctgttgtgtgactctggtaactagagatccctcagacccttttagtcagtgtggaaaatctctagcagtggcgcccgaacagggacttgaaagcgaaagggaaaccagaggagctctctcgacgcaggactcggcttgctgaagcgcgcacggcaagaggcgaggggcggcgactggtgagtacgccaaaaattttgactagcggaggctagaaggagagagatgggtgcgagagcgtcagtattaagcgggggagaattagatcgcgatgggaaaaaattcggttaaggccagggggaaagaaaaaatataaattaaaacatatagtatgggcaagcagggagctagaacgattcgcagttaatcctggcctgttagaaacatcagaaggctgtagacaaatactgggacagctacaaccatcccttcagacaggatcagaagaacttagatcattatataatacagtagcaaccctctattgtgtgcatcaaaggatagagataaaagacaccaaggaagctttagacaagatagaggaagagcaaaacaaaagtaagaccaccgcacagcaagcggccgctgatcttcagacctggaggaggagatatgagggacaattggagaagtgaattatataaatataaagtagtaaaaattgaaccattaggagtagcacccaccaaggcaaagagaagagtggtgcagagagaaaaaagagcagtgggaataggagctttgttccttgggttcttgggagcagcaggaagcactatgggcgcagcgtcaatgacgctgacggtacaggccagacaattattgtctggtatagtgcagcagcagaacaatttgctgagggctattgaggcgcaacagcatctgttgcaactcacagtctggggcatcaagcagctccaggcaagaatcctggctgtggaaagatacctaaaggatcaacagctcctggggatttggggttgctctggaaaactcatttgcaccactgctgtgccttggaatgctagttggagtaataaatctctggaacagatttggaatcacacgacctggatggagtgggacagagaaattaacaattacacaagcttaatacactccttaattgaagaatcgcaaaaccagcaagaaaagaatgaacaagaattattggaattagataaatgggcaagtttgtggaattggtttaacataacaaattggctgtggtatataaaattattcataatgatagtaggaggcttggtaggtttaagaatagtttttgctgtactttctatagtgaatagagttaggcagggatattcaccattatcgtttcagacccacctcccaaccccgaggggacccgacaggcccgaaggaatagaagaagaaggtggagagagagacagagacagatccattcgattagtgaacggatctcgacggtatcggttaacttttaaaagaaaaggggggattggggggtacagtgcaggggaaagaatagtagacataatagcaacagacatacaaactaaagaattacaaaaacaaattacaaaaattcaaaattttccgataagcttgggagttccgcgttacataacttacggtaaatggcccgcctggctgaccgcccaacgacccccgcccattgacgtcaataatgacgtatgttcccatagtaacgccaatagggactttccattgacgtcaatgggtggagtatttacggtaaactgcccacttggcagtacatcaagtgtatcatatgccaagtacgccccctattgacgtcaatgacggtaaatggcccgcctggcattatgcccagtacatgaccttatgggactttcctacttggcagtacatctacgtattagtcatcgctattaccatggtgatgcggttttggcagtacatcaatgggcgtggatagcggtttgactcacggggatttccaagtctccaccccattgacgtcaatgggagtttgttttggcaccaaaatcaacgggactttccaaaatgtcgtaacaactccgccccattgacgcaaatgggcggtaggcgtgtacggtgggaggtctatataagcagagctcgtttagtgaaccgtcagatcgcctggagacgccatccacgctgttttgacctccatagaagacaccgactctagaactagtggatcccccgggctgcaggaattcgtcgactggatccggtaccgaggagatctgccgccgcgatcgccggcgcgccagatctcaagcttaactagttagcggaccgacgcgtacgcggccgctcgagatgagcgggggcgaggagctgttcgccggcatcgtgcccgtgctgatcgagctggacggcgacgtgcacggccacaagttcagcgtgcgcggcgagggcgagggcgacgccgactacggcaagctggagatcaagttcatctgcaccaccggcaagctgcccgtgccctggcccaccctggtgaccaccctctgctacggcatccagtgcttcgcccgctaccccgagcacatgaagatgaacgacttcttcaagagcgccatgcccgagggctacatccaggagcgcaccatccagttccaggacgacggcaagtacaagacccgcggcgaggtgaagttcgagggcgacaccctggtgaaccgcatcgagctgaagggcaaggacttcaaggaggacggcaacatcctgggccacaagctggagtacagcttcaacagccacaacgtgtacatccgccccgacaaggccaacaacggcctggaggctaacttcaagacccgccacaacatcgagggcggcggcgtgcagctggccgaccactaccagaccaacgtgcccctgggcgacggccccgtgctgatccccatcaaccactacctgagcactcagaccaagatcagcaaggaccgcaacgaggcccgcgaccacatggtgctcctggagtccttcagcgcctgctgccacacccacggcatggacgagctgtacaggtccggactcagataagtttaaacccgatatcatcatctagggcggccaattccgcccctctccccccccctaacgttactggccgaagccgcttggaataaggccggtgtgcgtttgtctatatgttattttccaccatattgccgtcttttggcaatgtgagggcccggaaacctggccctgtcttcttgacgagcattcctaggggtctttcccctctcgccaaaggaatgcaaggtctgttgaatgtcgtgaaggaagcagttcctctggaagcttcttgaagacaaacaacgtctgtagcgaccctttgcaggcagcggaaccccccacctggcgacaggtgcctctgcggccaaaagccacgtgtataagatacacctgcaaaggcggcacaaccccagtgccacgttgtgagttggatagttgtggaaagagtcaaatggctctcctcaagcgtattcaacaaggggctgaaggatgcccagaaggtaccccattgtatgggatctgatctggggcctcggtgcacatgctttacatgtgtttagtcgaggttaaaaaaacgtctaggccccccgaaccacggggacgtggttttcctttgaaaaacacgatgataagcttgccacaacccacaaggagacgaccttccatgaccgagtacaagcccacggtgcgcctcgccacccgcgacgacgtcccccgggccgtacgcaccctcgccgccgcgttcgccgactaccccgccacgcgccacaccgtcgacccggaccgccacatcgagcgggtcaccgagctgcaagaactcttcctcacgcgcgtcgggctcgacatcggcaaggtgtgggtcgcggacgacggcgccgcggtggcggtctggaccacgccggagagcgtcgaagcgggggcggtgttcgccgagatcggcccgcgcatggccgagttgagcggttcccggctggccgcgcagcaacagatggaaggcctcctggcgccgcaccggcccaaggagcccgcgtggttcctggccaccgtcggcgtctcgcccgaccaccagggcaagggtctgggcagcgccgtcgtgctccccggagtggaggcggccgagcgcgccggggtgcccgccttcctggagacctccgcgccccgcaacctccccttctacgagcggctcggcttcaccgtcaccgccgacgtcgaggtgcccgaaggaccgcgcacctggtgcatgacccgcaagcccggtgcctgaaattagatcgataccgtcgacaatcaacctctggattacaaaatttgtgaaagattgactggtattcttaactatgttgctccttttacgctatgtggatacgctgctttaatgcctttgtatcatgctattgcttcccgtatggctttcattttctcctccttgtataaatcctggttgctgtctctttatgaggagttgtggcccgttgtcaggcaacgtggcgtggtgtgcactgtgtttgctgacgcaacccccactggttggggcattgccaccacctgtcagctcctttccgggactttcgctttccccctccctattgccacggcggaactcatcgccgcctgccttgcccgctgctggacaggggctcggctgttgggcactgacaattccgtggtgttgtcggggaagctgacgtcctttccatggctgctcgcctgtgttgccacctggattctgcgcgggacgtccttctgctacgtcccttcggccctcaatccagcggaccttccttcccgcggcctgctgccggctctgcggcctcttccgcgtcttcgccttcgccctcagacgagtcggatctccctttgggccgcctccccgcctgaatacgagctcggtacctttaagaccaatgacttacaaggcagctgtagatcttagccactttttaaaagaaaaggggggactggaagggctaattcactcccaacgaagacaagatctgctttttgcttgtactgggtctctctggttagaccagatctgagcctgggagctctctggctaactagggaacccactgcttaagcctcaataaagcttgccttgagtgcttcaagtagtgtgtgcccgtctgttgtgtgactctggtaactagagatccctcagacccttttagtcagtgtggaaaatctctagcagtagtagttcatgtcatcttattattcagtatttataacttgcaaagaaatgaatatcagagagtgagaggaacttgtttattgcagcttataatggttacaaataaagcaatagcatcacaaatttcacaaataaagcatttttttcactgcattctagttgtggtttgtccaaactcatcaatgtatcttatcatgtctggctctagctatcccgcccctaactccgcccatcccgcccctaactccgcccagttccgcccattctccgccccatggctgactaattttttttatttatgcagaggccgaggccgcctcggcctctgagctattccagaagtagtgaggaggcttttttggaggcctagggacgtacccaattcgccctatagtgagtcgtattacgcgcgctcactggccgtcgttttacaacgtcgtgactgggaaaaccctggcgttacccaacttaatcgccttgcagcacatccccctttcgccagctggcgtaatagcgaagaggcccgcaccgatcgcccttcccaacagttgcgcagcctgaatggcgaatgggacgcgccctgtagcggcgcattaagcgcggcgggtgtggtggttacgcgcagcgtgaccgctacacttgccagcgccctagcgcccgctcctttcgctttcttcccttcctttctcgccacgttcgccggctttccccgtcaagctctaaatcgggggctccctttagggttccgatttagtgctttacggcacctcgaccccaaaaaacttgattagggtgatggttcacgtagtgggccatcgccctgatagacggtttttcgccctttgacgttggagtccacgttctttaatagtggactcttgttccaaactggaacaacactcaaccctatctcggtctattcttttgatttataagggattttgccgatttcggcctattggttaaaaaatgagctgatttaacaaaaatttaacgcgaattttaacaaaatattaacgtttacaatttcccaggtggcacttttcggggaaatgtgcgcggaacccctatttgtttatttttctaaatacattcaaatatgtatccgctcatgagacaataaccctgataaatgcttcaataatattgaaaaaggaagagtatgagtattcaacatttccgtgtcgcccttattcccttttttgcggcattttgccttcctgtttttgctcacccagaaacgctggtgaaagtaaaagatgctgaagatcagttgggtgcacgagtgggttacatcgaactggatctcaacagcggtaagatccttgagagttttcgccccgaagaacgttttccaatgatgagcacttttaaagttctgctatgtggcgcggtattatcccgtattgacgccgggcaagagcaactcggtcgccgcatacactattctcagaatgacttggttgagtactcaccagtcacagaaaagcatcttacggatggcatgacagtaagagaattatgcagtgctgccataaccatgagtgataacactgcggccaacttacttctgacaacgatcggaggaccgaaggagctaaccgcttttttgcacaacatgggggatcatgtaactcgccttgatcgttgggaaccggagctgaatgaagccataccaaacgacgagcgtgacaccacgatgcctgtagcaatggcaacaacgttgcgcaaactattaactggcgaactacttactctagcttcccggcaacaattaatagactggatggaggcggataaagttgcaggaccacttctgcgctcggcccttccggctggctggtttattgctgataaatctggagccggtgagcgtgggtctcgcggtatcattgcagcactggggccagatggtaagccctcccgtatcgtagttatctacacgacggggagtcaggcaactatggatgaacgaaatagacagatcgctgagataggtgcctcactgattaagcattggtaactgtcagaccaagtttactcatatatactttagattgatttaaaacttcatttttaatttaaaaggatctaggtgaagatcctttttgataatctcatgaccaaaatcccttaacgtgagttttcgttccactgagcgtcagaccccgtagaaaagatcaaaggatcttcttgagatcctttttttctgcgcgtaatctgctgcttgcaaacaaaaaaaccaccgctaccagcggtggtttgtttgccggatcaagagctaccaactctttttccgaaggtaactggcttcagcagagcgcagataccaaatactgtccttctagtgtagccgtagttaggccaccacttcaagaactctgtagcaccgcctacatacctcgctctgctaatcctgttaccagtggctgctgccagtggcgataagtcgtgtcttaccgggttggactcaagacgatagttaccggataaggcgcagcggtcgggctgaacggggggttcgtgcacacagcccagcttggagcgaacgacctacaccgaactgagatacctacagcgtgagctatgagaaagcgccacgcttcccgaagggagaaaggcggacaggtatccggtaagcggcagggtcggaacaggagagcgcacgagggagcttccagggggaaacgcctggtatctttatagtcctgtcgggtttcgccacctctgacttgagcgtcgatttttgtgatgctcgtcaggggggcggagcctatggaaaaacgccagcaacgcggcctttttacggttcctggccttttgctggccttttgctcacatgttctttcctgcgttatcccctgattctgtggataaccgtattaccgcctttgagtgagctgataccgctcgccgcagccgaacgaccgagcgcagcgagtcagtgagcgaggaagcggaagagcgcccaatacgcaaaccgcctctccccgcgcgttggccgattcattaatgcagctggcacgacaggtttcccgactggaaagcgggcagtgagcgcaacgcaattaatgtgagttagctcactcattaggcaccccaggctttacactttatgcttccggctcgtatgttgtgtggaattgtgagcggataacaatttcacacaggaaacagctatgaccatgattacgccaagcgcgcaattaaccctcactaaagggaacaaaagctggagctgcaagctt

SEQ ID NO: 190 - protein, 220 aa, synthetic construct
  REGION 1..220: note = Synthetic peptide
  VARIANT 143: note = Xaa can be any naturally occurring amino acid
MASAGMQILGVVLTLLGWVNGLVSCALPMWKVTAFIGNSIVVAQVVWEGLWMSCVVQSTGQMQCKVYDSLLALPQDLQAARALCVIALLVALFGLLVYLAGAKCTTCVEEKDSKARLVLTSGIVFVISGVLTLIPVCWTAHAXIRDFYNPLVAEAQKRELGASLYLGWAASGLLLLGGGLLCCTCPSGGSQGPSHYMARYSTSAPAISRGPSEYPTKNYV

SEQ ID NO: 191 - DNA, 68 bp, synthetic construct
  misc_feature 1..68: note = Synthetic polynucleotide
  source 1..68: mol_type = other DNA
cagaaactcatctcagaagaggatctggcagcaaatgatatcctggattacaaggatgacgacgataa

SEQ ID NO: 192 - DNA, 683 bp, Homo sapiens
  misc_feature 1..683: note = REGION - NCBI / NM_021195.4, 2017-06-04
  source 1..683: mol_type = genomic DNA
ccgcgatcgccatggcctctgccggaatgcagatcctgggagtcgtcctgacactgctgggctgggtgaatggcctggtctcctgtgccctgcccatgtggaaggtgaccgctttcatcggcaacagcatcgtggtggcccaggtggtgtgggagggcctgtggatgtcctgcgtggtgcagagcaccggccagatgcagtgcaaggtgtacgactcactgctggcgctgccacaggacctgcaggctgcacgtgccctctgtgtcatcgccctccttgtggccctgttcggcttgctggtctaccttgctggggccaagtgtaccacctgtgtggaggagaaggattccaaggcccgcctggtgctcacctctgggattgtctttgtcatctcaggggtcctgacgctaatccccgtgtgctggacggcgcatgccgtcatccgggacttctataaccccctggtggctgaggcccaaaagcgggagctgggggcctccctctacttgggctgggcggcctcaggccttttgttgctgggtggggggttgctgtgctgcacttgcccctcgggggggtcccagggccccagccattacatggcccgctactcaacatctgcccctgccatctctcgggggccctctgagtaccctaccaagaattacgtcacgcgtacgcgg

SEQ ID NO: 193 - DNA, 677 bp, Mus musculus
  misc_feature 1..677: note = REGION - NCBI / NM_018777.4, 2017-08-07
  source 1..677: mol_type = genomic DNA
gccgcgatcgccatggcctctactggtctgcaaatcttggggatcgtcctgaccctgcttggctgggtcaacgccctggtgtcctgtgccctgcccatgtggaaggtgaccgccttcatcggcaacagcatcgtcgtggcccagatggtgtgggaggggctgtggatgtcctgtgtggttcagagcactggccagatgcagtgcaaggtgtatgactcactgttggcgctgccccaggacctgcaggctgccagagccctctgtgttgtcaccctcctcattgtcctgcttggcctgctcgtgtacctggctggagccaagtgcactacctgtgtggaagataggaactccaagtctcgtctggtgctcatctctggcatcatctttgtcatttctggggtcctgacgctcattcctgtctgctggactgcccactctatcatccaggacttctacaaccccttggtggctgatgctcaaaagcgggagctgggggcctccctctacctgggctgggcagcctcaggccttttgctgctgggtggagggctactatgctgcgcctgctcttctggagggacccagggacccagacattacatggcctgctattctacatctgtcccacattctcggggaccctccgaatatcccaccaagaattatgtgacgcgtac

SEQ ID NO: 194 - DNA, 683 bp, synthetic construct
  misc_feature 1..683: note = Synthetic polynucleotide
  source 1..683: mol_type = other DNA
cgcgatcgccatggcctctgccggaatgcagatcctgggagtcgtcctgacactgctgggctgggtgaatggcctggtctcctgtgccctgcccatgtggaaggtgaccgctttcatcggcaacagcatcgtggtggcccaggtggtgtgggagggcctgtggatgtcctgcgtggtgcagagcaccggccagatgcagtgcaaggtgtacgactcactgctggcgctgccacaggacctgcaggctgcacgtgccctctgtgtcatcgccctccttgtggccctgttcggcttgctggtctaccttgctggggccaagtgtaccacctgtgtggaggagaaggattccaaggcccgcctggtgctcacctctgggattgtctttgtcatctcaggggtcctgacgctaatccccgtgtgctggacggcgcatgccatcatccgggacttctataaccccctggtggctgaggcccaaaagcgggagctgggggcctccctctacttgggctgggcggcctcaggccttttgttgctgggtggggggttgctgtgctgcacttgcccctcgggggggtcccagggccccagccattacatggcccgctactcaacatctgcccctgccatctctcgggggccctctgagtaccctaccaagaattacgtcacgcgtacgcggc

SEQ ID NO: 195 - DNA, 672 bp, Homo sapiens
  misc_feature 1..672: note = REGION - NCBI / NM_020982.3, 2017-04-15
  source 1..672: mol_type = genomic DNA
gccgcgatcgccatggcttcgaccggcttagaactgctgggcatgaccctggctgtgctgggctggctggggaccctggtgtcctgcgccctgcccctgtggaaggtgaccgccttcatcggcaacagcatcgtggtggcccaggtggtgtgggagggcctgtggatgtcctgcgtggtgcagagcacgggccagatgcagtgcaaggtgtacgactcactgctggctctgccgcaggacctgcaggccgcacgtgccctctgtgtcattgccctcctgctggccctgcttggcctcctggtggccatcacaggtgcccagtgtaccacgtgtgtggaggacgaaggtgccaaggcccgtatcgtgctcaccgcgggggtcatcctcctcctcgccggcatcctggtgctcatccctgtgtgctggacggcgcacgccatcatccaggacttctacaaccccctggtggctgaggccctcaagcgggagctgggggcctccctctacctgggctgggcggcggctgcactgcttatgctgggcggggggctcctctgctgcacgtgccccccgccccaggtcgagcggccccgcggacctcggctgggctactccatcccctcccgctcgggtgcatctggactggacaagagggactacgtgacgcgtacg

SEQ ID NO: 196 - DNA, 651 bp, Homo sapiens
  misc_feature 1..651: note = REGION - NCBI / NM_001305.4, 2017-07-10
  source 1..651: mol_type = genomic DNA
ccgcgatcgccatggcctccatggggctacaggtaatgggcatcgcgctggccgtcctgggctggctggccgtcatgctgtgctgcgcgctgcccatgtggcgcgtgacggccttcatcggcagcaacattgtcacctcgcagaccatctgggagggcctatggatgaactgcgtggtgcagagcaccggccagatgcagtgcaaggtgtacgactcgctgctggcactgccgcaggacctgcaggcggcccgcgccctcgtcatcatcagcatcatcgtggctgctctgggcgtgctgctgtccgtggtggggggcaagtgtaccaactgcctggaggatgaaagcgccaaggccaagaccatgatcgtggcgggcgtggtgttcctgttggccggccttatggtgatagtgccggtgtcctggacggcccacaacatcatccaagacttctacaatccgctggtggcctccgggcagaagcgggagatgggtgcctcgctctacgtcggctgggccgcctccggcctgctgctccttggcggggggctgctttgctgcaactgtccaccccgcacagacaagccttactccgccaagtattctgctgcccgctctgctgctgccagcaactacgtgacgcgtacgcggc

SEQ ID NO: 197 - DNA, 680 bp, Homo sapiens
  misc_feature 1..680: note = REGION - NCBI / NM_001306.3, 2017-07-10
  source 1..680: mol_type = genomic DNA
gccgcgatcgccatgtccatgggcctggagatcacgggcaccgcgctggccgtgctgggctggctgggcaccatcgtgtgctgcgcgttgcccatgtggcgcgtgtcggccttcatcggcagcaacatcatcacgtcgcagaacatctgggagggcctgtggatgaactgcgtggtgcagagcaccggccagatgcagtgcaaggtgtacgactcgctgctggcactgccacaggaccttcaggcggcccgcgccctcatcgtggtggccatcctgctggccgccttcgggctgctagtggcgctggtgggcgcccagtgcaccaactgcgtgcaggacgacacggccaaggccaagatcaccatcgtggcaggcgtgctgttccttctcgccgccctgctcaccctcgtgccggtgtcctggtcggccaacaccattatccgggacttctacaaccccgtggtgcccgaggcgcagaagcgcgagatgggcgcgggcctgtacgtgggctgggcggccgcggcgctgcagctgctggggggcgcgctgctctgctgctcgtgtcccccacgcgagaagaagtacacggccaccaaggtcgtctactccgcgccgcgctccaccggcccgggagccagcctgggcacaggctacgaccgcaaggactacgtcacgcgtac

SEQ ID NO: 198 - protein, 214 aa, synthetic construct
  REGION 1..214: note = Synthetic peptide
DIVLTQSPATLSVTPGNSVSLSCRASQSIGGNLHWYQQKSHESPRLLIKYASQSISGIPSRFSGSGSGTDFTLSINSVETEDFGMYFCQQSNSWPYTFGGGTKLEIKRADAAPTVSIFPPSSEQLTSGGASVVCFLNNFYPKDINVKWKIDGSERQNGVLNSWTDQDSKDSTYSMSSTLTLTKDEYERHNSYTCEATHKTSTSPIVKSFNRNEC

SEQ ID NO: 199 - protein, 444 aa, synthetic construct
  REGION 1..444: note = Synthetic peptide
DVQLQESGPSLVKPSQTLSLTCSVTGDSITSDYWSWIRKFPGNRLEYMGYVSYSGSTYYNPSLKSRISITRDTSKNQYYLDLNSVTTEDTATYYCANWDGDYWGQGTLVTVSSAAKTTAPSVYPLAPVCGDTTGSSVTLGCLVKGYFPEPVTLTWNSGSLSSGVHTFPAVLQSDLYTLSSSVTVTSSTWPSQSITCNVAHPASSTKVDKKIEPRGPTIKPCPPCKCPAPNLLGGPSVFIFPPKIKDVLMISLSPIVTCVVVDVSEDDPDVQISWFVNNVEVHTAQTQTHREDYNSTLRVVSALPIQHQDWMSGKEFKCKVNNKDLPAPIERTISKPKGSVRAPQVYVLPPPEEEMTKKQVTLTCMVTDFMPEDIYVEWTNNGKTELNYKNTEPVLDSDGSYFMYSKLRVEKKNWVERNSYSCSVVHEGLHNHHTTKSFSRTPGK

SEQ ID NO: 200 - protein, 220 aa, synthetic construct; identical to SEQ ID NO: 190
  REGION 1..220: note = Synthetic peptide
  VARIANT 143: note = Xaa can be any naturally occurring amino acid

SEQ ID NO: 201 - protein, 220 aa, synthetic construct; identical to SEQ ID NO: 190
  REGION 1..220: note = Synthetic peptide
  VARIANT 143: note = Xaa can be any naturally occurring amino acid

SEQ ID NO: 202-207 - skipped (6 entries)

SEQ ID NO: 208 - DNA, 21 bp, synthetic construct
  misc_feature 1..21: note = Synthetic polynucleotide
  source 1..21: mol_type = other DNA
tccagtgtaagttccacttac

SEQ ID NO: 209 - skipped

SEQ ID NO: 210 - DNA, 27 bp, synthetic construct
  misc_feature 1..27: note = Synthetic polynucleotide
  source 1..27: mol_type = other DNA
caccagtatcatcgttccccgctcacg

SEQ ID NO: 211 - DNA, 24 bp, synthetic construct
  misc_feature 1..24: note = Synthetic polynucleotide
  source 1..24: mol_type = other DNA
ggctacacctttactacctacacg

SEQ ID NO: 212 - DNA, 24 bp, synthetic construct
  misc_feature 1..24: note = Synthetic polynucleotide
  source 1..24: mol_type = other DNA
attaatcctagcagtggatatact

SEQ ID NO: 213 - DNA, 27 bp, synthetic construct
  misc_feature 1..27: note = Synthetic polynucleotide
  source 1..27: mol_type = other DNA
gcaaacggggattactacgtcgcttac

SEQ ID NO: 214 - DNA, 18 bp, synthetic construct
  misc_feature 1..18: note = Synthetic polynucleotide
  source 1..18: mol_type = other DNA
gagaatatttacagttat

SEQ ID NO: 215 - skipped

SEQ ID NO: 216 - DNA, 27 bp, synthetic construct
  misc_feature 1..27: note = Synthetic polynucleotide
  source 1..27: mol_type = other DNA
caacatcattatactgttccgtggacg

SEQ ID NO: 217 - DNA, 24 bp, synthetic construct
  misc_feature 1..24: note = Synthetic polynucleotide
  source 1..24: mol_type = other DNA
ggtttcactttcagtgattactgg

SEQ ID NO: 218 - DNA, 30 bp, synthetic construct
  misc_feature 1..30: note = Synthetic polynucleotide
  source 1..30: mol_type = other DNA
attagattgaaatctgataattatgcaaca

SEQ ID NO: 219 - DNA, 24 bp, synthetic construct
  misc_feature 1..24: note = Synthetic polynucleotide
  source 1..24: mol_type = other DNA
aatgatggccccccctcggggtgt

SEQ ID NO: 220 - DNA, 18 bp, synthetic construct
  misc_feature 1..18: note = Synthetic polynucleotide
  source 1..18: mol_type = other DNA
gagaatatttacagttat

SEQ ID NO: 221 - skipped

SEQ ID NO: 222 - DNA, 27 bp, synthetic construct
  misc_feature 1..27: note = Synthetic polynucleotide
  source 1..27: mol_type = other DNA
caacatcattatactgttccgtggacg

SEQ ID NO: 223 - DNA, 24 bp, synthetic construct
  misc_feature 1..24: note = Synthetic polynucleotide
  source 1..24: mol_type = other DNA
ggattcactttcagtaattactgg

SEQ ID NO: 224 - DNA, 30 bp, synthetic construct; identical to SEQ ID NO: 218
  misc_feature 1..30: note = Synthetic polynucleotide
  source 1..30: mol_type = other DNA

SEQ ID NO: 225 - DNA, 24 bp, synthetic construct
  misc_feature 1..24: note = Synthetic polynucleotide
  source 1..24: mol_type = other DNA
aatgatggccccccctcggggtgt

SEQ ID NO: 226 - DNA, 33 bp, synthetic construct
  misc_feature 1..33: note = Synthetic polynucleotide
  source 1..33: mol_type = other DNA
cagagccttgtacacagtgatggaaacacctat

SEQ ID NO: 227 - skipped

SEQ ID NO: 228 - DNA, 27 bp, synthetic construct
  misc_feature 1..27: note = Synthetic polynucleotide
  source 1..27: mol_type = other DNA
tctcaaagtacacatgttccttacacg

SEQ ID NO: 229 - DNA, 24 bp, synthetic construct
  misc_feature 1..24: note = Synthetic polynucleotide
  source 1..24: mol_type = other DNA
ggctacacctttactagctacacg

SEQ ID NO: 230 - DNA, 24 bp, synthetic construct
  misc_feature 1..24: note = Synthetic polynucleotide
  source 1..24: mol_type = other DNA
attaatcctagcagtacttatact

SEQ ID NO: 231 - DNA, 30 bp, synthetic construct
  misc_feature 1..30: note = Synthetic polynucleotide
  source 1..30: mol_type = other DNA
tcaagaggggaactgggagggtttgcttac

SEQ ID NO: 232 - DNA, 33 bp, synthetic construct
  misc_feature 1..33: note = Synthetic polynucleotide
  source 1..33: mol_type = other DNA
cagagcattgtacatagtaatggaaacacctat

SEQ ID NO: 233 - skipped

SEQ ID NO: 234 - DNA, 27 bp, synthetic construct
  misc_feature 1..27: note = Synthetic polynucleotide
  source 1..27: mol_type = other DNA
tttcaaggttcacatgttccattcacg

SEQ ID NO: 235 - DNA, 24 bp, synthetic construct
  misc_feature 1..24: note = Synthetic polynucleotide
  source 1..24: mol_type = other DNA
ggatacatattcactcactatatt

SEQ ID NO: 236 - DNA, 24 bp, synthetic construct
  misc_feature 1..24: note = Synthetic polynucleotide
  source 1..24: mol_type = other DNA
attaatccttacaatgatggtact

SEQ ID NO: 237 - DNA, 39 bp, synthetic construct
  misc_feature 1..39: note = Synthetic polynucleotide
  source 1..39: mol_type = other DNA
gcaagatactacggctacccttactattctatggactac

SEQ ID NO: 238 - DNA, 36 bp, synthetic construct
  misc_feature 1..36: note = Synthetic polynucleotide
  source 1..36: mol_type = other DNA
cagagtctgctcaacagtagaacccgaaagaactac

SEQ ID NO: 239 - skipped

SEQ ID NO: 240 - DNA, 24 bp, synthetic construct
  misc_feature 1..24: note = Synthetic polynucleotide
  source 1..24: mol_type = other DNA
aagcaatcttattatctgtacacg

SEQ ID NO: 241 - DNA, 27 bp, synthetic construct
  misc_feature 1..27: note = Synthetic polynucleotide
  source 1..27: mol_type = other DNA
ggctactccatcaccagtggttattac

SEQ ID NO: 242 - DNA, 21 bp, synthetic construct
  misc_feature 1..21: note = Synthetic polynucleotide
  source 1..21: mol_type = other DNA
atcagctacgatggtggcatt

SEQ ID NO: 243 - DNA, 30 bp, synthetic construct
  misc_feature 1..30: note = Synthetic polynucleotide
  source 1..30: mol_type = other DNA
gcaagatttggtaagggggctatggactac

SEQ ID NO: 244 - DNA, 21 bp, synthetic construct
  misc_feature 1..21: note = Synthetic polynucleotide
  source 1..21: mol_type = other DNA
tcaagtgtaagttccagttac

SEQ ID NO: 245 - skipped

SEQ ID NO: 246 - DNA, 27 bp, synthetic construct
  misc_feature 1..27: note = Synthetic polynucleotide
  source 1..27: mol_type = other DNA
caccagtatcatcgttccccacccacg

SEQ ID NO: 247 - DNA, 24 bp, synthetic construct
  misc_feature 1..24: note = Synthetic polynucleotide
  source 1..24: mol_type = other DNA
ggttactcattcactggctacacc

SEQ ID NO: 248 - DNA, 24 bp, synthetic construct
  misc_feature 1..24: note = Synthetic polynucleotide
  source 1..24: mol_type = other DNA
attaatccttacaatggtggtact

SEQ ID NO: 249 - DNA, 36 bp, synthetic construct
  misc_feature 1..36: note = Synthetic polynucleotide
  source 1..36: mol_type = other DNA
gcaagaggggtctatgattacgacggatttacttac

SEQ ID NO: 250 - DNA, 33 bp, synthetic construct; identical to SEQ ID NO: 226
  misc_feature 1..33: note = Synthetic polynucleotide
  source 1..33: mol_type = other DNA

SEQ ID NO: 251 - skipped

SEQ ID NO: 252 - DNA, 27 bp, synthetic construct
  misc_feature 1..27: note = Synthetic polynucleotide
  source 1..27: mol_type = other DNA
tctcaaagtacacatgttccttacacg

SEQ ID NO: 253 - DNA, 24 bp, synthetic construct
  misc_feature 1..24: note = Synthetic polynucleotide
  source 1..24: mol_type = other DNA
ggctacacctttactacctacacg

SEQ ID NO: 254 - DNA, 24 bp, synthetic construct
  misc_feature 1..24: note = Synthetic polynucleotide
  source 1..24: mol_type = other DNA
attaatcctcgcagtggttatagt

SEQ ID NO: 255 - DNA, 30 bp, synthetic construct; identical to SEQ ID NO: 231
  misc_feature 1..30: note = Synthetic polynucleotide
  source 1..30: mol_type = other DNA

SEQ ID NO: 256 - DNA, 18 bp, synthetic construct
  misc_feature 1..18: note = Synthetic polynucleotide
  source 1..18: mol_type = other DNA
cagaccattggtacatgg

SEQ ID NO: 257 - skipped

SEQ ID NO: 258 - DNA, 27 bp, synthetic construct
  misc_feature 1..27: note = Synthetic polynucleotide
  source 1..27: mol_type = other DNA
caacaactttacagtattcctcggacg

SEQ ID NO: 259 - DNA, 24 bp, synthetic construct
  misc_feature 1..24: note = Synthetic polynucleotide
  source 1..24: mol_type = other DNA
ggatacagattcactgactacaac

SEQ ID NO: 260 - DNA, 24 bp, synthetic construct
  misc_feature 1..24: note = Synthetic polynucleotide
  source 1..24: mol_type = other DNA
attaaccctaacaatggtggtact

SEQ ID NO: 261 - DNA, 30 bp, synthetic construct
  misc_feature 1..30: note = Synthetic polynucleotide
  source 1..30: mol_type = other DNA
gcaagagattacttgtacttctttgactgc

SEQ ID NO: 262 - DNA, 33 bp, synthetic construct
  misc_feature 1..33: note = Synthetic polynucleotide
  source 1..33: mol_type = other DNA
cagagccttgtacacagtaatggaaacacctat

SEQ ID NO: 263 - skipped

SEQ ID NO: 264 - DNA, 27 bp, synthetic construct
  misc_feature 1..27: note = Synthetic polynucleotide
  source 1..27: mol_type = other DNA
tctcaaattacacatgttccgtacacg

SEQ ID NO: 265 - DNA, 24 bp, synthetic construct
  misc_feature 1..24: note = Synthetic polynucleotide
  source 1..24: mol_type = other DNA
ggttataccttcacagactattca

SEQ ID NO: 266 - DNA, 24 bp, synthetic construct
  misc_feature 1..24: note = Synthetic polynucleotide
  source 1..24: mol_type = other DNA
ataagcactgagactggtgagcca

SEQ ID NO: 267 - DNA, 30 bp, synthetic construct
  misc_feature 1..30: note = Synthetic polynucleotide
  source 1..30: mol_type = other DNA
actagaggtctatggtcctcgtttgcttac

SEQ ID NO: 268 - DNA, 30 bp, synthetic construct
  misc_feature 1..30: note = Synthetic polynucleotide
  source 1..30: mol_type = other DNA
aaaagtgtcagtacatctggctatagttat

SEQ ID NO: 269 - skipped

SEQ ID NO: 270 - DNA, 27 bp, synthetic construct
  misc_feature 1..27: note = Synthetic polynucleotide
  source 1..27: mol_type = other DNA
cagcacagtagggagcttccgctcacg

SEQ ID NO: 271 - DNA, 24 bp, synthetic construct
  misc_feature 1..24: note = Synthetic polynucleotide
  source 1..24: mol_type = other DNA
ggattcactttcagtagctttgga

SEQ ID NO: 272 - DNA, 24 bp, synthetic construct
  misc_feature 1..24: note = Synthetic polynucleotide
  source 1..24: mol_type = other DNA
attagtagtgacagtaggaccatc

SEQ ID NO: 273 - DNA, 33 bp, synthetic construct
  misc_feature 1..33: note = Synthetic polynucleotide
  source 1..33: mol_type = other DNA
gcaagagactacggtagaacctacgaggcttac

SEQ ID NO: 274 - DNA, 18 bp, synthetic construct
  misc_feature 1..18: note = Synthetic polynucleotide
  source 1..18: mol_type = other DNA
caggacattggaggaaat

SEQ ID NO: 275 - skipped

SEQ ID NO: 276 - DNA, 27 bp, synthetic construct
  misc_feature 1..27: note = Synthetic polynucleotide
  source 1..27: mol_type = other DNA
ctacagcgtaatgcgtatccgctcact

SEQ ID NO: 277 - DNA, 24 bp, synthetic construct
  misc_feature 1..24: note = Synthetic polynucleotide
  source 1..24: mol_type = other DNA
ggattcactttcagtagttatgcc

SEQ ID NO: 278 - DNA, 21 bp, synthetic construct
  misc_feature 1..21: note = Synthetic polynucleotide
  source 1..21: mol_type = other DNA
attagaagtggtggtaccacc

SEQ ID NO: 279 - DNA, 36 bp, synthetic construct
  misc_feature 1..36: note = Synthetic polynucleotide
  source 1..36: mol_type = other DNA
gcaaaagtgggcggtaacccctatcctatggactac

SEQ ID NO: 280 - DNA, 21 bp, synthetic construct
  misc_feature 1..21: note = Synthetic polynucleotide
  source 1..21: mol_type = other DNA
tcaagtataagttccaattac

SEQ ID NO: 281 - skipped

SEQ ID NO: 282 - DNA, 27 bp, synthetic construct
  misc_feature 1..27: note = Synthetic polynucleotide
  source 1..27: mol_type = other DNA
cagcagggtagtagtataccgctcacg

SEQ ID NO: 283 - DNA, 24 bp, synthetic construct
  misc_feature 1..24: note = Synthetic polynucleotide
  source 1..24: mol_type = other DNA
ggatacgccttcagtaattacttg

SEQ ID NO: 284 - DNA, 24 bp, synthetic construct
  misc_feature 1..24: note = Synthetic polynucleotide
  source 1..24: mol_type = other DNA
attaatcctggaagtggtggtact

SEQ ID NO: 285 - DNA, 45 bp, synthetic construct
  misc_feature 1..45: note = Synthetic polynucleotide
  source 1..45: mol_type = other DNA
gcaagatcatacttcggtagaagctacccctatactatggactac

SEQ ID NO: 286 - DNA, 30 bp, synthetic construct
  misc_feature 1..30: note = Synthetic polynucleotide
  source 1..30: mol_type = other DNA
caaagtgttgattatgatggtgataattat

SEQ ID NO: 287 - skipped

SEQ ID NO: 288 - DNA, 27 bp, synthetic construct
  misc_feature 1..27: note = Synthetic polynucleotide
  source 1..27: mol_type = other DNA
cagcaaagtaatgaggatccattcacg

SEQ ID NO: 289 - DNA, 24 bp, synthetic construct
  misc_feature 1..24: note = Synthetic polynucleotide
  source 1..24: mol_type = other DNA
ggctacacattcactgattatgct

SEQ ID NO: 290 - DNA, 24 bp, synthetic construct
  misc_feature 1..24: note = Synthetic polynucleotide
  source 1..24: mol_type = other DNA
attagtacatactctggtaataca

SEQ ID NO: 291 - DNA, 39 bp, synthetic construct
  misc_feature 1..39: note = Synthetic polynucleotide
  source 1..39: mol_type = other DNA
gcaagaaggggcgattacagcctctatgctatggactac

SEQ ID NO: 292 - DNA, 36 bp, synthetic construct
  misc_feature 1..36: note = Synthetic polynucleotide
  source 1..36: mol_type = other DNA
caaagtgttttattcagttcaaatcagaaaaactac

SEQ ID NO: 293 - skipped

SEQ ID NO: 294 - DNA, 24 bp, synthetic construct
  misc_feature 1..24: note = Synthetic polynucleotide
  source 1..24: mol_type = other DNA
catcaatacctctcctcgcgcacg

SEQ ID NO: 295 - DNA, 24 bp, synthetic construct
  misc_feature 1..24: note = Synthetic polynucleotide
  source 1..24: mol_type = other DNA
ggattcactttcagtagctttgga

SEQ ID NO: 296 - DNA, 24 bp, synthetic construct
  misc_feature 1..24: note = Synthetic polynucleotide
  source 1..24: mol_type = other DNA
attagtagtgacagtaggaccatc

SEQ ID NO: 297 - DNA, 33 bp, synthetic construct; identical to SEQ ID NO: 273
  misc_feature 1..33: note = Synthetic polynucleotide
  source 1..33: mol_type = other DNA

SEQ ID NO: 298 - DNA, 30 bp, synthetic construct
  misc_feature 1..30: note = Synthetic polynucleotide
  source 1..30: mol_type = other DNA
gaaagtgttgataattatggcattagtttt

SEQ ID NO: 299 - skipped

SEQ ID NO: 300 - DNA, 27 bp, synthetic construct
  misc_feature 1..27: note = Synthetic polynucleotide
  source 1..27: mol_type = other DNA
cagcaaagtaaggaggttccgctcacg

SEQ ID NO: 301 - DNA, 24 bp, synthetic construct
  misc_feature 1..24: note = Synthetic polynucleotide
  source 1..24: mol_type = other DNA
ggattccctttcagtagctctgcc

SEQ ID NO: 302 - DNA, 21 bp, synthetic construct
  misc_feature 1..21: note = Synthetic polynucleotide
  source 1..21: mol_type = other DNA
attaatagtgatggtaacacc

SEQ ID NO: 303 - DNA, 39 bp, synthetic construct
  misc_feature 1..39: note = Synthetic polynucleotide
  source 1..39: mol_type = other DNA
acaagaaacggggactataggtacgacgagtttgcttac

SEQ ID NO: 304 - DNA, 21 bp, synthetic construct
  misc_feature 1..21: note = Synthetic polynucleotide
  source 1..21: mol_type = other DNA
tcaagtgtaagttccagttac

SEQ ID NO: 305 - skipped

SEQ ID NO: 306 - DNA, 27 bp, synthetic construct
  misc_feature 1..27: note = Synthetic polynucleotide
  source 1..27: mol_type = other DNA
caccagtatcatcgttccccacccacg

SEQ ID NO: 307 - DNA, 24 bp, synthetic construct
  misc_feature 1..24: note = Synthetic polynucleotide
  source 1..24: mol_type = other DNA
ggctacacctttactggctactgg

SEQ ID NO: 308 - DNA, 24 bp, synthetic construct
  misc_feature 1..24: note = Synthetic polynucleotide
  source 1..24: mol_type = other DNA
attaatcctagcactggttatact

SEQ ID NO: 309 - DNA, 36 bp, synthetic construct
  misc_feature 1..36: note = Synthetic polynucleotide
  source 1..36: mol_type = other DNA
gcaagagaggggattactactgtgctggttgactac

SEQ ID NO: 310 - DNA, 36 bp, synthetic construct; identical to SEQ ID NO: 292
  misc_feature 1..36: note = Synthetic polynucleotide
  source 1..36: mol_type = other DNA

SEQ ID NO: 311 - skipped

SEQ ID NO: 312 - DNA, 24 bp, synthetic construct
  misc_feature 1..24: note = Synthetic polynucleotide
  source 1..24: mol_type = other DNA
catcaatacctctcctcgcgcacg

SEQ ID NO: 313 - DNA, 24 bp, synthetic construct
  misc_feature 1..24: note = Synthetic polynucleotide
  source 1..24: mol_type = other DNA
ggttactctttcactggctacaat

SEQ ID NO: 314 - DNA, 24 bp, synthetic construct
  misc_feature 1..24: note = Synthetic polynucleotide
  source 1..24: mol_type = other DNA
attgatccttactatggtggttct

SEQ ID NO: 315 - DNA, 42 bp, synthetic construct
  misc_feature 1..42: note = Synthetic polynucleotide
  source 1..42: mol_type = other DNA
gcaagagagaggtcgggctacgttttctctgctatggactac

SEQ ID NO: 316 - DNA, 36 bp, synthetic construct; identical to SEQ ID NO: 292
  misc_feature 1..36: note = Synthetic polynucleotide
  source 1..36: mol_type = other DNA

SEQ ID NO: 317 - skipped

SEQ ID NO: 318 - DNA, 24 bp, synthetic construct
  misc_feature 1..24: note = Synthetic polynucleotide
  source 1..24: mol_type = other DNA
catcaatacctctcctcgcgcacg

SEQ ID NO: 319 - DNA, 24 bp, synthetic construct
  misc_feature 1..24: note = Synthetic polynucleotide
  source 1..24: mol_type = other DNA
ggttactcattcactggctacacc

SEQ ID NO: 320 - DNA, 24 bp, synthetic construct
  misc_feature 1..24: note = Synthetic polynucleotide
  source 1..24: mol_type = other DNA
attaatccttacaatggtgttact

SEQ ID NO: 321 - DNA, 48 bp, synthetic construct
  misc_feature 1..48: note = Synthetic polynucleotide
  source 1..48: mol_type = other DNA
acaagagatcccctttactacggctacagggactctactatggactac

SEQ ID NO: 322 - DNA, 33 bp, synthetic construct; identical to SEQ ID NO: 226
  misc_feature 1..33: note = Synthetic polynucleotide
  source 1..33: mol_type = other DNA

SEQ ID NO: 323 - skipped

SEQ ID NO: 324 - DNA, 27 bp, synthetic construct
  misc_feature 1..27: note = Synthetic polynucleotide
  source 1..27: mol_type = other DNA
tctcaaagtacacatgttccttacacg

SEQ ID NO: 325 - DNA, 24 bp, synthetic construct
  misc_feature 1..24: note = Synthetic polynucleotide
  source 1..24: mol_type = other DNA
ggctacacctttactagctacacg

SEQ ID NO: 326 - DNA, 24 bp, synthetic construct
  misc_feature 1..24: note = Synthetic polynucleotide
  source 1..24: mol_type = other DNA
attaatcctagcagtacgtatact

SEQ ID NO: 327 - DNA, 30 bp, synthetic construct; identical to SEQ ID NO: 231
  misc_feature 1..30: note = Synthetic polynucleotide
  source 1..30: mol_type = other DNA

SEQ ID NO: 328 - DNA, 18 bp, synthetic construct
  misc_feature 1..18: note = Synthetic polynucleotide
  source 1..18: mol_type = other DNA
cagggcattagaggtaat

SEQ ID NO: 329 - skipped

SEQ ID NO: 330 - DNA, 27 bp, synthetic construct
  misc_feature 1..27: note = Synthetic polynucleotide
  source 1..27: mol_type = other DNA
ctacagcgtaatgcgtatcctctcacg

SEQ ID NO: 331 - DNA, 24 bp, synthetic construct
  misc_feature 1..24: note = Synthetic polynucleotide
  source 1..24: mol_type = other DNA
ggattcactttcagtagttttgcc

SEQ ID NO: 332 - DNA, 21 bp, synthetic construct
  misc_feature 1..21: note = Synthetic polynucleotide
  source 1..21: mol_type = other DNA
attagaagtggtggtattacc

SEQ ID NO: 333 - DNA, 39 bp, synthetic construct
  misc_feature 1..39: note = Synthetic polynucleotide
  source 1..39: mol_type = other DNA
gcaagagttagtacggctacgtactatggtatggactac

SEQ ID NO: 334 - DNA, 325 bp, synthetic construct
  misc_feature 1..325: note = Synthetic polynucleotide
  source 1..325: mol_type = other DNA
caaattgttctcacccagtctccagcaatcatgtctgcatctctaggggaacgggtcaccatgacctgcactgccagctccagtgtaagttccacttactttcactggtaccaacagaagccaggatcctcccccaaactctggatttatagcacatccaacctggcttctggagtcccacgtcgcttcagtggcagtgcgtctgggacctcttactctctcacaatcagcagcatggaggctgaagatgctgccacttattattgccaccagtatcatcgttccccgctcacgttcggtgctgggaccaagctggagctgaaac

SEQ ID NO: 335 - DNA, 349 bp, synthetic construct
  misc_feature 1..349: note = Synthetic polynucleotide
  source 1..349: mol_type = other DNA
caggtccagctgcagcagtctgcagctgaactggcaagacctggggcctcagtgaagatgtcctgcaaggcttctggctacacctttactacctacacgatgcactgggtaaaacagaggcctggacagggtctggaatggattggattcattaatcctagcagtggatatactgactacaatcagaagttcaaggacaggaccacattgactgcagacaaatcctccagcacagtctacatgcaactgagtagcctgacatctgaggactctgcggtctattactgtgcaaacggggattactacgtcgcttactggggccaagggactctggtcactgtctctgcag

SEQ ID NO: 336 - DNA, 322 bp, synthetic construct
  misc_feature 1..322: note = Synthetic polynucleotide
  source 1..322: mol_type = other DNA
gacatccagatgactcagtctccagcctccctatctgcatctgtgggagaaactgtcaccatcacatgtcgaataagcgagaatatttacagttatttagcatggtatcagcagaaacagggaaaatctcctcagctcctggtctataatgcaaaaatcttagtagaaggtgtgccatcaaggttcagtggcagtggatcaggcacacagttttctctgaagatcaacagcctgcagcctgaagattttgggaattattactgtcaacatcattatactgttccgtggacgttcggtggaggcaccaaactggaaatcaaac

SEQ ID NO: 337 - DNA, 352 bp, synthetic construct
  misc_feature 1..352: note = Synthetic polynucleotide
  source 1..352: mol_type = other DNA
gaagtgaagcttgaggagtctggaggaggcttggtgcaacctggaggatccatgaaactctcctgtgttgcctctggtttcactttcagtgattactggatgaactgggtccgccagtctccagagaaggggcttgaatgggttgctcaaattagattgaaatctgataattatgcaacacattatgcggagtctgtgaaagggaggttcaccatctcaagagatgattccaaaagaagtgtctacctgcaaatgaacaacttaagggctgaagacactggaacttattactgcaatgatggccccccctcggggtgttggggccaaggcaccactctcatagtctcctcag

SEQ ID NO: 338 - DNA, 322 bp, synthetic construct
  misc_feature 1..322: note = Synthetic polynucleotide
  source 1..322: mol_type = other DNA
gacatccagatgactcagtctccagcctccctatctgcatctgtgggagaaactgtcaccatcacatgtcgaataagtgagaatatttacagttatttagcatggtatcagcagaaacagggaaaatctcctcagctcctggtctataatgcaaaaatcttagtagaaggtgtgccatcaaggttcagtggcagtggatcaggcacacagttttctctgaagatcaacagcctgcagcctgaagattttgggaattattactgtcaacatcattatactgttccgtggacgttcggtggaggcaccaaactggaaatcaaac

SEQ ID NO: 339 - DNA, 352 bp, synthetic construct
  misc_feature 1..352: note = Synthetic polynucleotide
  source 1..352: mol_type = other DNA
gaagtgaagcttgaggagtctggaggaggcttggtgcaacctggaggatccatgaaactctcctgtgttgcctctggattcactttcagtaattactggatgaactgggtccgccagtctccagagaaggggcttgaatgggttgctcaaattagattgaaatctgataattatgcaacacattatgcggagtctgtgaaagggaggttcaccatctcaagagatgattccaaaagaagtgtctacctgcaaatgaacaacttaagggctgaagacactggaacttattactgcaatgatggccccccctcggggtgttggggccaaggcaccactctcatagtctcctcag

SEQ ID NO: 340 - DNA, 337 bp, synthetic construct
  misc_feature 1..337: note = Synthetic polynucleotide
  source 1..337: mol_type = other DNA
gatgttgtgatgacccaaactccactctccctgcctgtcagtcttggagatcaagcctccatctcttgcagatctagtcagagccttgtacacagtgatggaaacacctatttaaattggtacctgcagaagccaggccagtctccaaagctcctgatctacaaagtttccaaccgtttttctggggtcccagacaggttcagtggcagtggatcagggacagatttcacactcaagatcaggagagtggaggctgaggatctgggagtttatttctgctctcaaagtacacatgttccttacacgttcggaggggggaccaagctggaaataaaac

SEQ ID NO: 341 - DNA, 352 bp, synthetic construct
  misc_feature 1..352: note = Synthetic polynucleotide
  source 1..352: mol_type = other DNA
caggtccagttgcagcagtctggggctgaactggcaagacctggggcctcagtgaagatgtcctgcaaggcttctggctacacctttactagctacacgatgcactggataaaacagagacctggacagggtcaggaatggattggatacattaatcctagcagtacttatactcattacattaagaaattcaaggacaaggccacattgactgcagacaaatcctccagcacagcctacatgcaactgcgcagcctgacatctgaggactctgcagtctattactgttcaagaggggaactgggagggtttgcttactggggccaagggactctggtcactgtctctgcag

SEQ ID NO: 342 - DNA, 337 bp, synthetic construct
  misc_feature 1..337: note = Synthetic polynucleotide
  source 1..337: mol_type = other DNA
gatgttttgatgacccaaactccactctccctgcctgtcagtcttggagatcaaccctccatctcttgcagatctagtcagagcattgtacatagtaatggaaacacctatttagattggtacctgcagaaaccaggccagtctccaaagctcctgatctacaaagtttccaaccgattttctggggtcccagacaggttcagtggcagtggatcagggacagatttcacactcaagatcagcagagtggaggctgaggatctgggagtttattactgctttcaaggttcacatgttccattcacgttcggctcggggacaaggttggaaataaaac

SEQ ID NO: 343 - DNA, 361 bp, synthetic construct
  misc_feature 1..361: note = Synthetic polynucleotide
  source 1..361: mol_type = other DNA
gaagtccagctgcagcagtctggacctgagctggtaaagcctggggcttcagtgaagatgtcctgcaaggcttctggatacatattcactcactatattatgcactgggtgaagcagaagcctgggcagggccttgagtggattggatgtattaatccttacaatgatggtactaagtacaatgagaagttcaaaggcaaggccacactgacttcagacaaatcctccagcacagcctacatggagctcagcagcctgacctctgaggactctgcggtctattactgtgcaagatactacggctacccttactattctatggactactggggtcaaggaacctcagtcaccgtctcctcag

SEQ ID NO: 344 - DNA, 337 bp, synthetic construct
  misc_feature 1..337: note = Synthetic polynucleotide
  source 1..337: mol_type = other DNA
gccattgtgatgttccagtctccatcctccctggttgtgtcagcaggagagaaggtcactatgagctgcaaatccagtcagagtctgctcaacagtagaacccgaaagaactacttggcttggtaccagcagaaaccagggcagtctcctaaactgctgatctactgggcatccactagggaatctggggtccctgatcgcttcacaggcagtggatctgggacagatttcactctcaccatcagcagtgtgcaggctgaagacctggcagtttattactgcaagcaatcttattatctgtacacgttcggaggggggaccaagctggaaataaaac

SEQ ID NO: 345 - DNA, 352 bp, synthetic construct
  misc_feature 1..352: note = Synthetic polynucleotide
  source 1..352: mol_type = other DNA
gatgtgcagcttcaggagtcaggacctggcctcgtgaaatcttctcagtctctgtctctcacctgctctgtcactggctactccatcaccagtggttattactggaaatggatccggcagtttccaggaaacaaactggaatggatgggctacatcagctacgatggtggcattaactacaacccatctctcaaaaatcgaatctccatcactcgtgacacatctaagaaccagtttttcctgaagttgaattctgtgactactgaggacacagccaaatattactgtgcaagatttggtaagggggctatggactactggggtcaaggaacctcagtcaccgtctcctcag

SEQ ID NO: 346 - DNA, 325 bp, synthetic construct
  misc_feature 1..325: note = Synthetic polynucleotide
  source 1..325: mol_type = other DNA
caaattgttctcacccagtctccagcaatcatgtctgcatctctgggggaccgggtcaccatgacctgcactgccagctcaagtgtaagttccagttacttgcactggtaccagcagaagccaggatcctcccccaaactctggatttatagcacatccaacctggcttctggagtcccagctcgcttcagtggcagtgggtctgggacctcttactctctcacaatcagcagcatggaggctgaagatgctgccacttattactgccaccagtatcatcgttccccacccacgttcggctcggggacaaagttggaaataaaac

SEQ ID NO: 347 - DNA, 358 bp, synthetic construct
  misc_feature 1..358: note = Synthetic polynucleotide
  source 1..358: mol_type = other DNA
gaggtccagctgcaacagtctggacctgagctggtgaagcctggagcttcaatgaagatatcctgcaaggcttctggttactcattcactggctacaccatgaactgggtgaagcagagccatggaaagaaccttgagtggattggacttattaatccttacaatggtggtactaactacaaccagaagttcaagggcaaggccacattaactgtagacaagtcatccagcacagcctacatggagctcctcagtctgacatctgaggactctgcagtctattactgtgcaagaggggtctatgattacgacggatttacttactggggccaagggactctggtcactgtctctgcag

SEQ ID NO: 348 - DNA, 337 bp, synthetic construct
  misc_feature 1..337: note = Synthetic polynucleotide
  source 1..337: mol_type = other DNA
gatgttgtgatgacccaaactccactctccctgcctgtcagtcttggagatcaagcctccatctcttgcagatctagtcagagccttgtacacagtgatggaaacacctatttatattggtacctgcagaagccaggccagtctccaaagctcctgatctacaaagtttccaaccgattttctggggtcccagacaggttcagtggcagtggatcagggacagatttcacactcaagatcagcagagtggaggctgaggatctgggagtttatttctgctctcaaagtacacatgttccttacacgttcggaggggggaccaagctggaaataaaac

SEQ ID NO: 349 - DNA, 352 bp, synthetic construct
  misc_feature 1..352: note = Synthetic polynucleotide
  source 1..352: mol_type = other DNA
caggtccagctgcagcagtctggggctgaactggcaagacctggggcctcagtgaagatgtcctgcaaggcttctggctacacctttactacctacacgatgcactggttaaaacagaggcctggacagggtctggaatggattggatacattaatcctcgcagtggttatagtaattacaatcagaagttcaaggacaaggccacattgactgcagacaagtcctccaacacagcctacatgcaactgaacaccctgacatctgaggactctaaagtctattactgttcaagaggggaactgggagggtttgcttactggggccaagggactctggtcactgtctctgcag

SEQ ID NO: 350 - DNA, 322 bp, synthetic construct
  misc_feature 1..322: note = Synthetic polynucleotide
  source 1..322: mol_type = other DNA
gacattcagatgacccagtctcctgcctcccagtctgcatctctgggagaaagtgtcaccatcacatgcctggcaagtcagaccattggtacatggttagcatggtatcagcagaaaccagggaaatctcctcagctcctgatttatgctgcagccagcttggcagatggggtcccatcaaggttcagtggtagtggatctggcacaagattttctttcaagatcagcagcctacaggctgaagattttgtaagttattactgtcaacaactttacagtattcctcggacgttcggtggaggcaccaagctggaaatcaaac

SEQ ID NO: 351 - DNA, 352 bp, synthetic construct
  misc_feature 1..352: note = Synthetic polynucleotide
  source 1..352: mol_type = other DNA
gaggtccagctgcaacagtctggacctgagctggtgaagcctggggcttcagtgaagatgtcctgcaaggcttctggatacagattcactgactacaacatgcactgggtgaagcagagccatggaaagagccttgagtggattggatatattaaccctaacaatggtggtactaactacaaccaaaacttcaagggcaaggccacattgactgtgaacaagtcctccagcacagcctacatggagctccgcagcctgacatcggaggattctgcagcctattactgtgcaagagattacttgtacttctttgactgctggggccaaggcaccactctcacagtctcctcag

SEQ ID NO: 352 - DNA, 337 bp, synthetic construct
  misc_feature 1..337: note = Synthetic polynucleotide
  source 1..337: mol_type = other DNA
gatgttgtgatgacccaaactccactctccctgcctgtcagtcttggagatcaagcctccatctcttgcagagctagtcagagccttgtacacagtaatggaaacacctatttacattggttcctgcagaagccaggccagtctccaaagctcctgatctacaaagtttccaaccgattttctggggtcccagacaggttcagtggcagtggatcacggacagatttcacactcaagatcagcagagtggaggctgaggatctgggagtttatttctgctctcaaattacacatgttccgtacacgttcggaggggggaccaagctggaaataaaac

SEQ ID NO: 353 - DNA, 352 bp, synthetic construct
  misc_feature 1..352: note = Synthetic polynucleotide
  source 1..352: mol_type = other DNA
caaatccagttggtgcagtctggacctgcgctgaagaagcctggagagacagtcaagatctcctgcaaggcttctggttataccttcacagactattcaatgcactggataaagcaggctccaggaaagggtttaaagtggatgggctggataagcactgagactggtgagccaacatatgcagatggcttcaagggacggtttgacttctctttggaaacctctgccgacactgcctatttgtccatcaacaacctcacaaatgaggacacggctacatatttctgtactagaggtctatggtcctcgtttgcttactggggccaagggactctggtcactgtctctgcag

SEQ ID NO: 354 - DNA, 334 bp, synthetic construct
  misc_feature 1..334: note = Synthetic polynucleotide
  source 1..334: mol_type = other DNA
gacattgtgctgacacagtctcctgcttccttagctgtatctctggggcagagggccaccatctcatgcagggccagcaaaagtgtcagtacatctggctatagttatatacactggtaccaacagaaaccaggacagccacccaaactcctcatctatcttgcatccaacctagaatctggggtccctgccaggttcagtggcagtgggtctgggacagacttcaccctcaacatccatcctgtggaggaggaggatgctgcaacctattactgtcagcacagtagggagcttccgctcacgttcggtgctgggaccaagctggagctgaaac

SEQ ID NO: 355 - DNA, 355 bp, synthetic construct
  misc_feature 1..355: note = Synthetic polynucleotide
  source 1..355: mol_type = other DNA
gatgtgcagctggtggagtctgggggaggcttggtgcagcctagagggtcccggaaactctcctgtgcagcctctggattcactttcagtagctttggaatgcactgggttcgtcaggctccagagaaggggctggagtgggtcgcatacattagtagtgacagtaggaccatctattatgcagacacagtgaagggccgattcaccatctccagagacaatcccacgaacaccctgttcctgcaaatgaccagtctcaggtctgaggacacggccatgtattactgtgcaagagactacggtagaacctacgaggcttactggggccaagggactctggtcactgtctctgcag

SEQ ID NO: 356 - DNA, 322 bp, synthetic construct
  misc_feature 1..322: note = Synthetic polynucleotide
  source 1..322: mol_type = other DNA
gacatccagatgattcagtctccatcgtccatgtttgcctctctgggagacagagtcagtctctcttgtcgggctagtcaggacattggaggaaatttagactggtatcagcagaaaccaggtggaactattaaactcctgatctactccacatccaatttaaattctggtgtcccatcaaggttcagtggcagtgggtctgggtcagattattctctcaccatcaccagcctggagtctgaagattttgcagactattactgtctacagcgtaatgcgtatccgctcactttcggtgctgggaccaagctggagctgaaac

SEQ ID NO: 357 - DNA, 355 bp, synthetic construct
  misc_feature 1..355: note = Synthetic polynucleotide
  source 1..355: mol_type = other DNA
gaagtgaaactgatggagtctgggggagacttagtgaagcctggagggtccctgaaactctcctgtgcagcctctggattcactttcagtagttatgccatgtcttgggttcgccagactccagagaagaggctggagtgggtcgcgtccattagaagtggtggtaccacctactatccagacagtgtgaagggccgattcaccatctccagagataatgccaggaacatcctgtacctgcgaatgagtagtctgaggtctgaggacacggccatatattactgtgcaaaagtgggcggtaacccctatcctatggactactggggtcaaggaacctcagtcaccgtctcctcag

SEQ ID NO: 358 - DNA, 325 bp, synthetic construct
  misc_feature 1..325: note = Synthetic polynucleotide
  source 1..325: mol_type = other DNA
gaaattgtgctcacccagtctccaaccaccatggctgcatctcccggggagaagatcactatcacctgcagtgccagctcaagtataagttccaattacttgcattggtatcagcagaagccaggattctcccctaaactcttgatttataggacatccaatctggcttctggagtcccagctcgcttcagtggcagtgggtctgggacctcttactctctcacaattggcaccatggaggctgaagatgttgccacttactactgccagcagggtagtagtataccgctcacgttcggtgctgggaccaagctggagctgaaac

SEQ ID NO: 359 - DNA, 367 bp, synthetic construct
  misc_feature 1..367: note = Synthetic polynucleotide
  source 1..367: mol_type = other DNA
caggtccagctgcagcagtctggagctgagctggtaaggcctgggacttcagtgaaggtgtcctgcaaggcttctggatacgccttcagtaattacttgatagagtgggttaagcagaggcctggacagggccttgagtggattggagtgattaatcctggaagtggtggtactaactacaatgagaagttcaagggcaaggcaacaatgactgcagacaaatcctccagcactgcctacatgcacctcagcaacctgacatctgaggactctgtggtctatttctgtgcaagatcatacttcggtagaagctacccctatactatggactactggggtcaaggaacctcagtcaccgtctcctcag

SEQ ID NO: 360 - DNA, 334 bp, synthetic construct
  misc_feature 1..334: note = Synthetic polynucleotide
  source 1..334: mol_type = other DNA
gatattgtgctgacccaatctccagcttctttggctgtgtctctagggcagagggccaccatctcctgcaaggccagccaaagtgttgattatgatggtgataattatgtgaactggtaccaacagaaagtaggacagccacccaaactcctcatctctgctgcatccaatctagaatctgggatcccagccaggtttagtggcagtgggtctgggacagacttcaccctcaacatccatcctgtggaggaggaggatgctgcaacctattactgtcagcaaagtaatgaggatccattcacgttcggctcggggacaaagttggaaataaaac

SEQ ID NO: 361 - DNA, 361 bp, synthetic construct
  misc_feature 1..361: note = Synthetic polynucleotide
  source 1..361: mol_type = other DNA
caggtccagctgcagcagtctgggcctgagctggtgaggcctggggtctcagtgaagatttcctgcaagggttccggctacacattcactgattatgctatgcactgggtgaagcagagtcatgcaaagagtctagagtggattggagttattagtacatactctggtaatacaaactacaaccagaagtttcaggacaaggccaccatgactgtagacaaatcctccagcacagcctatatggcacttgccagattgacatctgacgattctgccatctattactgtgcaagaaggggcgattacagcctctatgctatggactactggggtcaaggaacctcagtcaccgtctcctcag

SEQ ID NO: 362 - DNA, 337 bp, synthetic construct
  misc_feature 1..337: note = Synthetic polynucleotide
  source 1..337: mol_type = other DNA
aacattatgatgacacagtcgccatcatctctggctgtgtctgcaggagaaaaggtcactatgagctgtaagtccagtcaaagtgttttattcagttcaaatcagaaaaactacttggcctggtaccagcagaaaccagggcagtctcctagactgctgatctactgggcatccactagggaatctggtgtccctgatcgcttcacaggcagtggatctgggacagattttactcttaccatcagcaatgttcaagctgaagacctggcagtttattactgtcatcaatacctctcctcgcgcacgttcggtgctgggaccaagctggagctgaaac

SEQ ID NO: 363 - DNA, 355 bp, synthetic construct; identical to SEQ ID NO: 355
  misc_feature 1..355: note = Synthetic polynucleotide
  source 1..355: mol_type = other DNA

SEQ ID NO: 364 - DNA, 334 bp, synthetic construct
  misc_feature 1..334: note = Synthetic polynucleotide
  source 1..334: mol_type = other DNA
gacattgtgctgacccaatctccagcttctttggctctgtctctagggcagagggccaccatctcctgcagagccagcgaaagtgttgataattatggcattagttttatgaactggttccaacagaaacccggacagccacccaaactcctcatctatgctgcatccaaccaaggatccggggtccctgccaggtttagtggcagtgggtctgggacagacttcagcctcaacatccatcctatggaggaggatgatactgcaatgtatttctgtcagcaaagtaaggaggttccgctcacgttcggtgctgggaccaagctggagctgaaac

SEQ ID NO: 365 - DNA, 358 bp, synthetic construct
  misc_feature 1..358: note = Synthetic polynucleotide
  source 1..358: mol_type = other DNA
gaagtgaggctggtggagtctgggggaggcttgatgcagcctggagggtccctgaaactcccctgtgcagcctctggattccctttcagtagctctgccatgtcttgggttcgccagactccagagaagaggctggagtgggtcgcatccattaatagtgatggtaacacctactatcccgacagtgtgaagggccgattcaccatctccagagatagtgccaggaacatcctgtacctccaaatgagcagtctgaggtctgaggacacggccatgtattactgtacaagaaacggggactataggtacgacgagtttgcttactggggccaagggactctggtcactgtctctgcag

SEQ ID NO: 366 - DNA, 325 bp, synthetic construct
  misc_feature 1..325: note = Synthetic polynucleotide
  source 1..325: mol_type = other DNA
caaattgttctcacccagtctccagcaatcatgtctgcatctctaggggaacgggtcaccatgacctgcactgccagctcaagtgtaagttccagttacttgcactggtaccagcagaagccaggatcctcccccaaactctggatttatagcacatccaacctggcttctggagtcccagctcgcttcagtggcagtgggtctgggacctcttactctctcacaatcagcagcatggaggctgaagatgctgccacttattactgccaccagtatcatcgttccccacccacgttcggagctgggaccaagctggagctgaaac

SEQ ID NO: 367 - DNA, 358 bp, synthetic construct
  misc_feature 1..358: note = Synthetic polynucleotide
  source 1..358: mol_type = other DNA
caggtccagcttcagcagtctggggctgaactggcaaaacctggggcctcagtgaagatgtcctgcaaggcttctggctacacctttactggctactggatgcactgggtaaaacagaggcctggacagggtctggaatggcttggatacattaatcctagcactggttatactgagtccaatcagaagttcaaggacaaggccacattgactgcagacaaatcctccaccacagcctacatgcaactgagaagcctgacacctgaggactctgcagtctattactgtgcaagagaggggattactactgtgctggttgactactggggccaaggcaccactctcacagtctcctcag

SEQ ID NO: 368 - DNA, 337 bp, synthetic construct; identical to SEQ ID NO: 362
  misc_feature 1..337: note = Synthetic polynucleotide
  source 1..337: mol_type = other DNA

SEQ ID NO: 369 - DNA, 364 bp, synthetic construct
  misc_feature 1..364: note = Synthetic polynucleotide
  source 1..364: mol_type = other DNA
caggtgcagctgaagcagtctggacctgagctggagaagcctggcgcttcagtgaagatatcctgcaaggcttctggttactctttcactggctacaatatgaactgggtgaagcagagcaatggaaagagccttgagtggattggaaatattgatccttactatggtggttctacctacaaccagaagttcacgggcaaggccacattgactgtagacaaatcctccagcacagcctacatgcagctcaagagcctgacatctgaggactctgcagtgtattactgtgcaagagagaggtcgggctacgttttctctgctatggactactggggtcaaggaacctcagtcaccgtctcctcag

SEQ ID NO: 370 - DNA, 337 bp, synthetic construct; identical to SEQ ID NO: 362
  misc_feature 1..337: note = Synthetic polynucleotide
  source 1..337: mol_type = other DNA

SEQ ID NO: 371 - DNA, 370 bp, synthetic construct
  misc_feature 1..370: note = Synthetic polynucleotide
  source 1..370: mol_type = other DNA
gaggtccagctgcaacagtctggacctgagctggtgaagcctggaggttcaatgaagatatcctgcaaggcttctggttactcattcactggctacaccatgaactgggtgaagcggagccatggaaagaaccttgagtggattggacttattaatccttacaatggtgttactacctacaaccagaacttcaagggcaaggccacattagctgtagacaagtcatccagcacagcctacatggagctcctcggtctgacatctgaggactctgcagtctattactgtacaagagatcccctttactacggctacagggactctactatggactactggggtcaaggaacctcagtcaccgtctcctcag

SEQ ID NO: 372 - DNA, 337 bp, synthetic construct; identical to SEQ ID NO: 340
  misc_feature 1..337: note = Synthetic polynucleotide
  source 1..337: mol_type = other DNA

SEQ ID NO: 373 - DNA, 352 bp, synthetic construct
  misc_feature 1..352: note = Synthetic polynucleotide
  source 1..352: mol_type = other DNA
gaggtccagctgcagcagtctggggctgaactggcaagacctggggcctcagtgaagatgtcctgcaaggcttctggctacacctttactagctacacgatgcactggataaaacagagacctggacagggtcaggaatggattggatacattaatcctagcagtacgtatactcattacattaagaagttcaaggacaaggccacattgactgcagacaaatcctccagcacagcctacatgcaactgcgcagcctgacatctgaggactctgcagtctattactgttcaagaggggaactgggagggtttgcttactggggccaagggactctggtcactgtctctgcag

SEQ ID NO: 374 - DNA, 322 bp, synthetic construct
  misc_feature 1..322: note = Synthetic polynucleotide
  source 1..322: mol_type = other DNA
gacatccagatgattcagtctccatcgtccatgtttgcctctctgggagacagagtcagtctctcttgtcgggctagtcagggcattagaggtaatttagactggtatcagcagaaaccaggtggaactattaaactcctgatctactccacatccattttaaattctggtgtcccatcaaggttcagtggcagtgggtctgggtcagattattctctcaccatcaccagcctagagtctgaagattttgcagactattactgtctacagcgtaatgcgtatcctctcacgttcggttctgggaccaagctggagctgaaac

SEQ ID NO: 375 - DNA, 358 bp, synthetic construct
  misc_feature 1..358: note = Synthetic polynucleotide
  source 1..358: mol_type = other DNA
gaagtgaagttggtggagtctgggggaggcttaatgaagcctggagggtccctgaaactctcctgtgcggcctctggattcactttcagtagttttgccttgtcttgggttcgccagactccagagaagaggctggagtgggtcgcatccattagaagtggtggtattacctaccatgcagacagtgtgaagggccgattcaccatctccagagataatgccgggaacatcctgtacctgcaaatgaacagtctgaggtctgaggacacggccatgtatttctgtgcaagagttagtacggctacgtactatggtatggactactggggtcaaggaacctcagtcaccgtctcctcag

SEQ ID NO: 376 - protein, 116 aa, synthetic construct
  REGION 1..116: note = Synthetic peptide
QVQLVQSGAEVKKPGASVKVSCKASGYTFTTYTMHWVRQAPGQGLEWMGFINPSSGYTDYAQKFQGRVTMTRDTSTSTVYMELSSLRSEDTAVYYCARGDYYVAYWGQGTLVTVSS

SEQ ID NO: 377 - protein, 116 aa, synthetic construct
  REGION 1..116: note = Synthetic peptide
QVQLVQSGAEVKKPGASVKVSCKASGYTFTTYTMHWVRQAPGQGLEWMGFINPSSGYTDYAQKFQGRVTMTADTSTSTVYMELSSLRSEDTAVYYCANGDYYVAYWGQGTLVTVSS

SEQ ID NO: 378 - protein, 116 aa, synthetic construct
  REGION 1..116: note = Synthetic peptide
QVQLVQSGAEVKKPGASVKMSCKASGYTFTTYTMHWVRQAPGQGLEWIGFINPSSGYTDYAQKFQGRVTLTADTSTSTVYMELSSLRSEDTAVYYCANGDYYVAYWGQGTLVTVSS

SEQ ID NO: 379 - protein, 116 aa, synthetic construct
  REGION 1..116: note = Synthetic peptide
QVQLVQSGAEVKKPGASVKMSCKASGYTFTTYTMHWVRQAPGQGLEWIGFINPSSGYTDYAQKFQGRVTLTADKSTSTVYMELSSLRSEDTAVYYCANGDYYVAYWGQGTLVTVSS

SEQ ID NO: 380 - protein, 108 aa, synthetic construct
  REGION 1..108: note = Synthetic peptide
DIQMTQSPSSLSASVGDRVTITCTASSSVSSTYFHWYQQKPGKAPKLLIYSTSNLASGVPSRFSGSGSGTDFTLTISSLQPEDFATYYCHQYHRSPLTFGQGTKLEIK

SEQ ID NO: 381 - protein, 108 aa, synthetic construct
  REGION 1..108: note = Synthetic peptide
DIQMTQSPSSLSASVGDRVTITCTASSSVSSTYFHWYQQKPGKAPKLLIYSTSNLASGVPSRFSGSGSGTDYTLTISSLQPEDFATYYCHQYHRSPLTFGQGTKLEIK

SEQ ID NO: 382 - protein, 108 aa, synthetic construct
  REGION 1..108: note = Synthetic peptide
DIQLTQSPSSLSASVGDRVTMTCTASSSVSSTYFHWYQQKPGKAPKLLIYSTSNLASGVPSRFSGSGSGTDYTLTISSMQPEDAATYYCHQYHRSPLTFGQGTKLEIK

SEQ ID NO: 383 - protein, 108 aa, synthetic construct
  REGION 1..108: note = Synthetic peptide
DIQLTQSPSSLSASVGDRVTMTCTASSSVSSTYFHWYQQKPGKAPKLWIYSTSNLASGVPSRFSGSGSGTDYTLTISSMQPEDAATYYCHQYHRSPLTFGQGTKLEIK

SEQ ID NO: 384 - protein, 117 aa, synthetic construct
  REGION 1..117: note = Synthetic peptide
EVQLLESGGGLVQPGGSLRLSCAASGFTFSNYWMNWVRQAPGKGLEWVSQIRLKSDNYATHYADSVKGRFTISRDNSKNTLYLQMNSLRAEDTAVYYCAKGPPSGCWGQGTLVTVSS

SEQ ID NO: 385 - protein, 117 aa, synthetic construct
  REGION 1..117: note = Synthetic peptide
EVQLLESGGGLVQPGGSMRLSCAASGFTFSNYWMNWVRQAPGKGLEWVAQIRLKSDNYATHYADSVKGRFTISRDDSKNTVYLQMNSLRAEDTGVYYCNDGPPSGCWGQGTLLTVSS

SEQ ID NO: 386 - protein, 117 aa, synthetic construct
  REGION 1..117: note = Synthetic peptide
EVQLLESGGGLVQPGGSMRLSCAASGFTFSNYWMNWVRQAPGKGLEWVAQIRLKSDNYATHYADSVKGRFTISRDDSKNTVYLQMNSLRAEDTGVYYCNDGPPSGYWGQGTLLTVSS

SEQ ID NO: 387 - protein, 117 aa, synthetic construct
  REGION 1..117: note = Synthetic peptide
EVQLLESGGGLVQPGGSMRLSCAASGFTFSNYWMNWVRQAPGKGLEWVAQIRLKSDNYATHYADSVKGRFTISRDDSKNTVYLQMNSLRAEDTGVYYCNDGPPSGSWGQGTLLTVSS

SEQ ID NO: 388 - protein, 107 aa, synthetic construct
  REGION 1..107: note = Synthetic peptide
DIQMTQSPSSLSASVGDRVTITCRISENIYSYLAWYQQKPGKAPKLLIYNAKILVEGVPSRFSGSGSGTDFTLTISSLQPEDFATYYCQHHYTVPWTFGQGTKLEIK

SEQ ID NO: 389 - protein, 107 aa, synthetic construct
  REGION 1..107: note = Synthetic peptide
DIQMTQSPSSLSASVGDRVTITCRISENIYSYLAWYQQKPGKAPKLLVYNAKILVEGVPSRFSGSGSGTDFTLTISSLQPEDFGTYYCQHHYTVPWTFGQGTKLEIK

SEQ ID NO: 390 - protein, 107 aa, synthetic construct
  REGION 1..107: note = Synthetic peptide
DIQMTQSPSSLSASVGDRVTITCRISENIYSYLAWYQQKPGKAPKLLVYNAKSLVEGVPSRFSGSGSGTDFTLTISSLQPEDFGTYYCQHHYTVPWTFGQGTKLEIK

SEQ ID NO: 391 - protein, 117 aa, synthetic construct
  REGION 1..117: note = Synthetic peptide
QVQLVQSGAEVKKPGASVKVSCKASGYTFTSYTMHWVRQAPGQGLEWMGYINPSSTYTHYAQKFQGRVTMTRDTSTSTVYMELSSLRSEDTAVYYCARGELGGFAYWGQGTLVTVSS

SEQ ID NO: 392 - protein, 117 aa, synthetic construct
  REGION 1..117: note = Synthetic peptide
QVQLVQSGAEVKKPGASVKVSCKASGYTFTSYTMHWVRQAPGQGLEWMGYINPSSTYTHYAQKFQGRVTMTADTSTSTVYMELSSLRSEDTAVYYCSRGELGGFAYWGQGTLVTVSS

SEQ ID NO: 393 - protein, 117 aa, synthetic construct
  REGION 1..117: note = Synthetic peptide
QVQLVQSGAEVKKPGASVKMSCKASGYTFTSYTMHWIRQAPGQGLEWIGYINPSSTYTHYAQKFQGRATLTADTSTSTAYMELSSLRSEDTAVYYCSRGELGGFAYWGQGTLVTVSS

SEQ ID NO: 394 - protein, 117 aa, synthetic construct
  REGION 1..117: note = Synthetic peptide
QVQLVQSGAEVKKPGASVKMSCKASGYTFTSYTMHWIRQAPGQGQEWIGYINPSSTYTHYAQKFQGRATLTADTSTSTAYMELSSLRSEDTAVYYCSRGELGGFAYWGQGTLVTVSS

SEQ ID NO: 395 - protein, 117 aa, synthetic construct
  REGION 1..117: note = Synthetic peptide
QVQLVQSGAEVKKPGASVKMSCKASGYTFTSYTMHWIRQAPGQGLEWIGYINPSSTYTHYAQKFQGRATLTADKSTSTAYMELSSLRSEDTAVYYCSRGELGGFAYWGQGTLVTVSS

SEQ ID NO: 396 - protein, 117 aa, synthetic construct
  REGION 1..117: note = Synthetic peptide
QVQLVQSGAEVKKPGASVKMSCKASGYTFTSYTMHWIRQAPGQGQEWIGYINPSSTYTHYAQKFQGRATLTADKSTSTAYMELSSLRSEDTAVYYCSRGELGGFAYWGQGTLVTVSS

SEQ ID NO: 397 - protein, 112 aa, synthetic construct
  REGION 1..112: note = Synthetic peptide
DVVMTQSPLSLPVTLGQPASISCRSSQSLVHSDGNTYLNWFQQRPGQSPRRLIYKVSNRFSGVPDRFSGSGSGTDFTLKISRVEAEDVGVYYCSQSTHVPYTFGQGTKLEIK

SEQ ID NO: 398 - protein, 112 aa, synthetic construct
  REGION 1..112: note = Synthetic peptide
DVVMTQSPLSLPVTLGQPASISCRSSQSLVHSDGNTYLNWYQQRPGQSPRLLIYKVSNRFSGVPDRFSGSGSGTDFTLKISRVEAEDVGVYYCSQSTHVPYTFGQGTKLEIK

SEQ ID NO: 399 - protein, 112 aa, synthetic construct
  REGION 1..112: note = Synthetic peptide
DVVMTQSPLSLPVTLGQPASISCRSSQSLVHSEGNTYLNWYQQRPGQSPRLLIYKVSNRFSGVPDRFSGSGSGTDFTLKISRVEAEDVGVYYCSQSTHVPYTFGQGTKLEIK

SEQ ID NO: 400 - protein, 112 aa, synthetic construct
  REGION 1..112: note = Synthetic peptide
DVVMTQSPLSLPVTLGQPASISCRSSQSLVHSSGNTYLNWYQQRPGQSPRLLIYKVSNRFSGVPDRFSGSGSGTDFTLKISRVEAEDVGVYYCSQSTHVPYTFGQGTKLEIK

SEQ ID NO: 401 - protein, 112 aa, synthetic construct
  REGION 1..112: note = Synthetic peptide
DVVMTQSPLSLPVTLGQPASISCRSSQSLVHSEGSTYLNWYQQRPGQSPRLLIYKVSNRFSGVPDRFSGSGSGTDFTLKISRVEAEDVGVYYCSQSTHVPYTFGQGTKLEIK

SEQ ID NO: 402 - protein, 112 aa, synthetic construct
  REGION 1..112: note = Synthetic peptide
DVVMTQSPLSLPVTLGQPASISCRSSQSLVHSSGSTYLNWYQQRPGQSPRLLIYKVSNRFSGVPDRFSGSGSGTDFTLKISRVEAEDVGVYYCSQSTHVPYTFGQGTKLEIK

SEQ ID NO: 403 - protein, 117 aa, synthetic construct
  REGION 1..117: note = Synthetic peptide
QVQLVQSGAEVKKPGASVKVSCKASGYRFTDYNMHWVRQAPGQGLEWMGYINPNNGGTNYAQKFQGRVTMTRDTSTSTVYMELSSLRSEDTAVYYCARDYLYFFDCWGQGTLVTVSS

SEQ ID NO: 404 - protein, 117 aa, synthetic construct
  REGION 1..117: note = Synthetic peptide
QVQLVQSGAEVKKPGASVKVSCKASGYRFTDYNMHWVRQAPGQGLEWMGYINPNNGGTNYAQKFQGRVTMTVDTSTSTVYMELSSLRSEDTAVYYCARDYLYFFDCWGQGTLVTVSS

SEQ ID NO: 405 - protein, 117 aa, synthetic construct
  REGION 1..117: note = Synthetic peptide
QVQLVQSGAEVKKPGASVKMSCKASGYRFTDYNMHWVRQAPGQGLEWIGYINPNNGGTNYAQKFQGRATLTVDTSTSTAYMELSSLRSEDTAVYYCARDYLYFFDCWGQGTLLTVSS

SEQ ID NO: 406 - protein, 117 aa, synthetic construct
  REGION 1..117: note = Synthetic peptide
QVQLVQSGAEVKKPGASVKMSCKASGYRFTDYNMHWVRQAPGQGLEWIGYINPNNGGTNYAQKFQGRATLTVDKSTSTAYMELSSLRSEDTAVYYCARDYLYFFDCWGQGTLLTVSS

SEQ ID NO: 407 - protein, 117 aa, synthetic construct
  REGION 1..117: note = Synthetic peptide
QVQLVQSGAEVKKPGASVKMSCKASGYRFTDYNMHWVRQAPGQGLEWIGYINPNNGGTNYAQKFQGRATLTVNKSTSTAYMELSSLRSEDTAVYYCARDYLYFFDCWGQGTLLTVSS

SEQ ID NO: 408 - protein, 117 aa, synthetic construct
  REGION 1..117: note = Synthetic peptide
QVQLVQSGAEVKKPGASVKMSCKASGYRFTDYNMHWVRQAPGQGLEWIGYINPNNGGTNYAQKFQGRATLTVNTSTSTAYMELSSLRSEDTAVYYCARDYLYFFDCWGQGTLLTVSS

SEQ ID NO: 409 - protein, 107 aa, synthetic construct
  REGION 1..107: note = Synthetic peptide
DIQMTQSPSSLSASVGDRVTITCLASQTIGTWLAWYQQKPGKAPKLLIYAAASLADGVPSRFSGSGSGTDFTLTISSLQPEDFATYYCQQLYSIPRTFGQGTKLEIK

SEQ ID NO: 410 - protein, 107 aa, synthetic construct
  REGION 1..107: note = Synthetic peptide
DIQMTQSPSSLSASVGDRVTITCLASQTIGTWLAWYQQKPGKAPKLLIYAAASLADGVPSRFSGSGSGTDFTFTISSLQPEDFVTYYCQQLYSIPRTFGQGTKLEIK

SEQ ID NO: 411 - protein, 107 aa, synthetic construct
  REGION 1..107: note = Synthetic peptide
DIQMTQSPSSLSASVGDRVTITCRASQTIGTWLAWYQQKPGKAPKLLIYAAASLADGVPSRFSGSGSGTDFTFTISSLQPEDFVTYYCQQLYSIPRTFGQGTKLEIK

SEQ ID NO: 412 - protein, 118 aa, synthetic construct
  REGION 1..118: note = Synthetic peptide
EVQLVESGGGLVQPGGSLRLSCAASGFTFSSFGMHWVRQAPGKGLEWVSYISSDSRTIYYADSVKGRFTISRDNAKNSLYLQMNSLRAEDTAVYYCARDYGRTYEAYWGQGTLVTVSS

SEQ ID NO: 413 - protein, 118 aa, synthetic construct
  REGION 1..118: note = Synthetic peptide
EVQLVESGGGLVQPGGSLRLSCAASGFTFSSFGMHWVRQAPGKGLEWVAYISSDSRTIYYADSVKGRFTISRDNAKNSLYLQMNSLRAEDTAVYYCARDYGRTYEAYWGQGTLVTVSS

SEQ ID NO: 414 - protein, 111 aa, synthetic construct
  REGION 1..111: note = Synthetic peptide
DIVMTQSPDSLAVSLGERATINCRASKSVSTSGYSYIHWYQQKPGQPPKLLIYLASNLESGVPDRFSGSGSGTDFTLTISSLQAEDVAVYYCQHSRELPLTFGQGTKLEIK

SEQ ID NO: 415 - protein, 111 aa, synthetic construct
  REGION 1..111: note = Synthetic peptide
DIVLTQSPDSLAVSLGERATINCRASKSVSTSGYSYIHWYQQKPGQPPKLLIYLASNLESGVPDRFSGSGSGTDFTLTISSVQAEDVAVYYCQHSRELPLTFGQGTKLELK

SEQ ID NO: 416 - protein, 121 aa, synthetic construct
  REGION 1..121: note = Synthetic peptide
QVQLVQSGAEVKKPGASVKVSCKASGYSFTGYNMNWVRQAPGQGLEWMGNIDPYYGGSTYAQKFQGRVTMTRDTSTSTVYMELSSLRSEDTAVYYCARERSGYVFSAMDYWGQGTLVTVSS

SEQ ID NO: 417 - protein, 121 aa, synthetic construct
  REGION 1..121: note = Synthetic peptide
QVQLVQSGAEVKKPGASVKVSCKASGYSFTGYNMNWVRQAPGQGLEWMGNIDPYYGGSTYAQKFQGRVTMTVDTSTSTVYMELSSLRSEDTAVYYCARERSGYVFSAMDYWGQGTLVTVSS

SEQ ID NO: 418 - protein, 121 aa, synthetic construct
  REGION 1..121: note = Synthetic peptide
QVQLVQSGAEVKKPGASVKISCKASGYSFTGYNMNWVRQAPGQGLEWIGNIDPYYGGSTYAQKFQGRATLTVDTSTSTAYMELSSLRSEDTAVYYCARERSGYVFSAMDYWGQGTLVTVSS

SEQ ID NO: 419 - protein, 121 aa, synthetic construct
  REGION 1..121: note = Synthetic peptide
QVQLVQSGAEVKKPGASVKISCKASGYSFTGYNMNWVRQAPGQGLEWIGNIDPYYGGSTYAQKFQGRATLTVDKSTSTAYMELSSLRSEDTAVYYCARERSGYVFSAMDYWGQGTLVTVSS

SEQ ID NO: 420 - protein, 112 aa, synthetic construct
  REGION 1..112: note = Synthetic peptide
DIVMTQSPDSLAVSLGERATINCKSSQSVLFSSNQKNYLAWYQQKPGQPPKLLIYWASTRESGVPDRFSGSGSGTDFTLTISSLQAEDVAVYYCHQYLSSRTFGQGTKLEIK

SEQ ID NO: 421 - protein, 112 aa, synthetic construct
  REGION 1..112: note = Synthetic peptide
DIVMTQSPDSLAVSLGERVTMNCKSSQSVLFSSNQKNYLAWYQQKPGQPPKLLIYWASTRESGVPDRFSGSGSGTDFTLTISSVQAEDVAVYYCHQYLSSRTFGQGTKLEIK

SEQ ID NO: 422 - protein, 117 aa, synthetic construct
  REGION 1..117: note = Synthetic peptide
EVQLLESGGGLVQPGGSMRLSCAASGFTFSNYWMNWVRQAPGKGLEWVAQIRLKSDNYATHYADSVKGRFTISRDDSKNTVYLQMNSLRAEDTGVYYCNDGPPSGAWGQGTLLTVSS

SEQ ID NO: 423 - protein, 117 aa, synthetic construct
  REGION 1..117: note = Synthetic peptide
QVQLVQSGAEVKKPGASVKVSCKASGYTFTSYTMHWVRQAPGQGLEWMGYINPSSTYTHYIKKFKDRVTMTADTSTSTVYMELSSLRSEDTAVYYCSRGELGGFAYWGQGTLVTVSS

SEQ ID NO: 424 - protein, 117 aa, synthetic construct
  REGION 1..117: note = Synthetic peptide
QVQLVQSGAEVKKPGASVKMSCKASGYTFTSYTMHWIRQAPGQGLEWIGYINPSSTYTHYIKKFKDRATLTADTSTSTAYMELSSLRSEDTAVYYCSRGELGGFAYWGQGTLVTVSS

SEQ ID NO: 425 - protein, 117 aa, synthetic construct
  REGION 1..117: note = Synthetic peptide
QVQLVQSGAEVKKPGASVKMSCKASGYTFTSYTMHWIRQAPGQGQEWIGYINPSSTYTHYIKKFKDRATLTADTSTSTAYMELSSLRSEDTAVYYCSRGELGGFAYWGQGTLVTVSS

SEQ ID NO: 426 - protein, 117 aa, synthetic construct
  REGION 1..117: note = Synthetic peptide
QVQLVQSGAEVKKPGASVKMSCKASGYTFTSYTMHWIRQAPGQGLEWIGYINPSSTYTHYIKKFKDRATLTADKSTSTAYMELSSLRSEDTAVYYCSRGELGGFAYWGQGTLVTVSS

SEQ ID NO: 427 - protein, 117 aa, synthetic construct
  REGION 1..117: note = Synthetic peptide
QVQLVQSGAEVKKPGASVKMSCKASGYTFTSYTMHWIRQAPGQGQEWIGYINPSSTYTHYIKKFKDRATLTADKSTSTAYMELSSLRSEDTAVYYCSRGELGGFAYWGQGTLVTVSS

SEQ ID NO: 428 - protein, 116 aa, synthetic construct
  REGION 1..116: note = Synthetic peptide
  VARIANT 5: note = Xaa can be any naturally occurring amino acid
  VARIANT 8: note = Xaa can be any naturally occurring amino acid
  VARIANT 11..13: note = Xaa can be any naturally occurring amino acid
  VARIANT 20: note = Xaa can be any naturally occurring amino acid
  VARIANT 31: note = Xaa can be any naturally occurring amino acid
  VARIANT 33: note = Xaa can be any naturally occurring amino acid
  VARIANT 35: note = Xaa can be any naturally occurring amino acid
  VARIANT 38: note = Xaa can be any naturally occurring amino acid
  VARIANT 40: note = Xaa can be any naturally occurring amino acid
  VARIANT 48: note = Xaa can be any naturally occurring amino acid
  VARIANT 50: note = Xaa can be any naturally occurring amino acid
  VARIANT 55: note = Xaa can be any naturally occurring amino acid
  VARIANT 57: note = Xaa can be any naturally occurring amino acid
  VARIANT 59: note = Xaa can be any naturally occurring amino acid
  VARIANT 61: note = Xaa can be any naturally occurring amino acid
  VARIANT 65..68: note = Xaa can be any naturally occurring amino acid
  VARIANT 70: note = Xaa can be any naturally occurring amino acid
  VARIANT 72: note = Xaa can be any naturally occurring amino acid
  VARIANT 74..76: note = Xaa can be any naturally occurring amino acid
  VARIANT 79..80: note = Xaa can be any naturally occurring amino acid
  VARIANT 82: note = Xaa can be any naturally occurring amino acid
  VARIANT 87: note = Xaa can be any naturally occurring amino acid
  VARIANT 90..91: note = Xaa can be any naturally occurring amino acid
  VARIANT 98: note = Xaa can be any naturally occurring amino acid
  VARIANT 101: note = Xaa can be any naturally occurring amino acid
  VARIANT 116: note = Xaa can be any naturally occurring amino acid
QVQLXQSXAEXXXPGASVKXSCKASGYTFTXYXMXWVXQXPGQGLEWXGXINPSXGXTXYXQKFXXXXTXTXDXSXSTXXMXLSSLXSEXXAVYYCAXGDXYVAYWGQGTLVTVSX

SEQ ID NO: 429 - protein, 116 aa, synthetic construct
  REGION 1..116: note = Synthetic peptide
  VARIANT 20: note = Xaa can be any naturally occurring amino acid
  VARIANT 31: note = Xaa can be any naturally occurring amino acid
  VARIANT 35: note = Xaa can be any naturally occurring amino acid
  VARIANT 48: note = Xaa can be any naturally occurring amino acid
  VARIANT 50: note = Xaa can be any naturally occurring amino acid
  VARIANT 59: note = Xaa can be any naturally occurring amino acid
  VARIANT 67: note = Xaa can be any naturally occurring amino acid
  VARIANT 70: note = Xaa can be any naturally occurring amino acid
  VARIANT 74: note = Xaa can be any naturally occurring amino acid
  VARIANT 79: note = Xaa can be any naturally occurring amino acid
  VARIANT 98: note = Xaa can be any naturally occurring amino acid
  VARIANT 101: note = Xaa can be any naturally occurring amino acid
QVQLVQSGAEVKKPGASVKXSCKASGYTFTXYTMXWVRQAPGQGLEWXGXINPSSGYTXYAQKFQGXVTXTADXSTSTXYMELSSLRSEDTAVYYCAXGDXYVAYWGQGTLVTVSS

SEQ ID NO: 430 - protein, 108 aa, synthetic construct
  REGION 1..108: note = Synthetic peptide
  VARIANT 1: note = Xaa can be any naturally occurring amino acid
  VARIANT 3..4: note = Xaa can be any naturally occurring amino acid
  VARIANT 9..11: note = Xaa can be any naturally occurring amino acid
  VARIANT 15: note = Xaa can be any naturally occurring amino acid
  VARIANT 17: note = Xaa can be any naturally occurring amino acid
  VARIANT 21: note = Xaa can be any naturally occurring amino acid
  VARIANT 24: note = Xaa can be any naturally occurring amino acid
  VARIANT 27: note = Xaa can be any naturally occurring amino acid
  VARIANT 29: note = Xaa can be any naturally occurring amino acid
  VARIANT 32: note = Xaa can be any naturally occurring amino acid
  VARIANT 34..35: note = Xaa can be any naturally occurring amino acid
  VARIANT 43..44: note = Xaa can be any naturally occurring amino acid
  VARIANT 48: note = Xaa can be any naturally occurring amino acid
  VARIANT 51..56: note = Xaa can be any naturally occurring amino acid
  VARIANT 61: note = Xaa can be any naturally occurring amino acid
  VARIANT 67: note = Xaa can be any naturally occurring amino acid
  VARIANT 71..73: note = Xaa can be any naturally occurring amino acid
  VARIANT 79..81: note = Xaa can be any naturally occurring amino acid
  VARIANT 84: note = Xaa can be any naturally occurring amino acid
  VARIANT 90..91: note = Xaa can be any naturally occurring amino acid
  VARIANT 93..96: note = Xaa can be any naturally occurring amino acid
  VARIANT 101: note = Xaa can be any naturally occurring amino acid
  VARIANT 107: note = Xaa can be any naturally occurring amino acid
XIXXTQSPXXXSASXGXRVTXTCXASXSXSSXYXXWYQQKPGXXPKLXIYXXXXXXSGVPXRFSGSXSGTXXXLTISSXXXEDXATYYCXXYXXXXLTFGXGTKLEXK

SEQ ID NO: 431 - protein, 108 aa, synthetic construct
  REGION 1..108: note = Synthetic peptide
  VARIANT 4: note = Xaa can be any naturally occurring amino acid
  VARIANT 21: note = Xaa can be any naturally occurring amino acid
  VARIANT 32: note = Xaa can be any naturally occurring amino acid
  VARIANT 34: note = Xaa can be any naturally occurring amino acid
  VARIANT 48: note = Xaa can be any naturally occurring amino acid
  VARIANT 51: note = Xaa can be any naturally occurring amino acid
  VARIANT 53: note = Xaa can be any naturally occurring amino acid
  VARIANT 61: note = Xaa can be any naturally occurring amino acid
  VARIANT 67: note = Xaa can be any naturally occurring amino acid
  VARIANT 79: note = Xaa can be any naturally occurring amino acid
  VARIANT 84: note = Xaa can be any naturally occurring amino acid
  VARIANT 91: note = Xaa can be any naturally occurring amino acid
  VARIANT 93: note = Xaa can be any naturally occurring amino acid
DIQXTQSPSSLSASVGDRVTXTCTASSSVSSXYXHWYQQKPGKAPKLXIYXTXNLASGVPXRFSGSXSGTDYTLTISSXQPEDXATYYCHXYXRSPLTFGQGTKLEIK

SEQ ID NO: 432 - protein, 117 aa, synthetic construct
  REGION 1..117: note = Synthetic peptide
  VARIANT 3: note = Xaa can be any naturally occurring amino acid
  VARIANT 5: note = Xaa can be any naturally occurring amino acid
  VARIANT 18..19: note = Xaa can be any naturally occurring amino acid
  VARIANT 23: note = Xaa can be any naturally occurring amino acid
  VARIANT 31: note = Xaa can be any naturally occurring amino acid
  VARIANT 33: note = Xaa can be any naturally occurring amino acid
  VARIANT 35: note = Xaa can be any naturally occurring amino acid
  VARIANT 40: note = Xaa can be any naturally occurring amino acid
  VARIANT 42: note = Xaa can be any naturally occurring amino acid
  VARIANT 49..50: note = Xaa can be any naturally occurring amino acid
  VARIANT 52..59: note = Xaa can be any naturally occurring amino acid
  VARIANT 61: note = Xaa can be any naturally occurring amino acid
  VARIANT 64: note = Xaa can be any naturally occurring amino acid
  VARIANT 76: note = Xaa can be any naturally occurring amino acid
  VARIANT 79..81: note = Xaa can be any naturally occurring amino acid
  VARIANT 87: note = Xaa can be any naturally occurring amino acid
  VARIANT 94..95: note = Xaa can be any naturally occurring amino acid
  VARIANT 99: note = Xaa can be any naturally occurring amino acid
  VARIANT 106: note = Xaa can be any naturally occurring amino acid
  VARIANT 112: note = Xaa can be any naturally occurring amino acid
  VARIANT 114: note = Xaa can be any naturally occurring amino acid
EVXLXESGGGLVQPGGSXXLSCXASGFTFSXYXMXWVRQXPXKGLEWVXXIXXXXXXXXTXYAXSVKGRFTISRDXSKXXXYLQMNXLRAEDTXXYYCXDGPPSGXWGQGTXLXVSS

SEQ ID NO: 433 - protein, 117 aa, synthetic construct
  REGION 1..117: note = Synthetic peptide
  VARIANT 31: note = Xaa can be any naturally occurring amino acid
  VARIANT 35: note = Xaa can be any naturally occurring amino acid
  VARIANT 50: note = Xaa can be any naturally occurring amino acid
  VARIANT 55: note = Xaa can be any naturally occurring amino acid
  VARIANT 79: note = Xaa can be any naturally occurring amino acid
  VARIANT 99: note = Xaa can be any naturally occurring amino acid
  VARIANT 106: note = Xaa can be any naturally occurring amino acid
EVQLLESGGGLVQPGGSMRLSCAASGFTFSXYWMXWVRQAPGKGLEWVAXIRLKXDNYATHYADSVKGRFTISRDDSKXTVYLQMNSLRAEDTGVYYCXDGPPSGXWGQGTLLTVSS

SEQ ID NO: 434 - protein, 107 aa, synthetic construct
  REGION 1..107: note = Synthetic peptide
  VARIANT 9: note = Xaa can be any naturally occurring amino acid
  VARIANT 17..18: note = Xaa can be any naturally occurring amino acid
  VARIANT 25: note = Xaa can be any naturally occurring amino acid
  VARIANT 27..28: note = Xaa can be any naturally occurring amino acid
  VARIANT 30: note = Xaa can be any naturally occurring amino acid
  VARIANT 34: note = Xaa can be any naturally occurring amino acid
  VARIANT 40: note = Xaa can be any naturally occurring amino acid
  VARIANT 43: note = Xaa can be any naturally occurring amino acid
  VARIANT 45: note = Xaa can be any naturally occurring amino acid
  VARIANT 48: note = Xaa can be any naturally occurring amino acid
  VARIANT 50: note = Xaa can be any naturally occurring amino acid
  VARIANT 52..53: note = Xaa can be any naturally occurring amino acid
  VARIANT 55..56: note = Xaa can be any naturally occurring amino acid
  VARIANT 70: note = Xaa can be any naturally occurring amino acid
  VARIANT 72: note = Xaa can be any naturally occurring amino acid
  VARIANT 74: note = Xaa can be any naturally occurring amino acid
  VARIANT 76: note = Xaa can be any naturally occurring amino acid
  VARIANT 84..85: note = Xaa can be any naturally occurring amino acid
  VARIANT 90..91: note = Xaa can be any naturally occurring amino acid
  VARIANT 93..94: note = Xaa can be any naturally occurring amino acid
  VARIANT 97: note = Xaa can be any naturally occurring amino acid
  VARIANT 100: note = Xaa can be any naturally occurring amino acid
DIQMTQSPXSLSASVGXXVTITCRXSXXIXSYLXWYQQKXGKXPXLLXYXAXXLXXGVPSRFSGSGSGTXFXLXIXSLQPEDFXXYYCQXXYXXPWXFGXGTKLEIK

SEQ ID NO: 435 - protein, 107 aa, synthetic construct
  REGION 1..107: note = Synthetic peptide
  VARIANT 25: note = Xaa can be any naturally occurring amino acid
  VARIANT 34: note = Xaa can be any naturally occurring amino acid
  VARIANT 48: note = Xaa can be any naturally occurring amino acid
  VARIANT 53: note = Xaa can be any naturally occurring amino acid
  VARIANT 55: note = Xaa can be any naturally occurring amino acid
  VARIANT 84..85: note = Xaa can be any naturally occurring amino acid
  VARIANT 90: note = Xaa can be any naturally occurring amino acid
  VARIANT 93: note = Xaa can be any naturally occurring amino acid
DIQMTQSPSSLSASVGDRVTITCRXSENIYSYLXWYQQKPGKAPKLLXYNAKXLXEGVPSRFSGSGSGTDFTLTISSLQPEDFXXYYCQXHYXVPWTFGQGTKLEIK

SEQ ID NO: 436 - protein, 117 aa, synthetic construct
  REGION 1..117: note = Synthetic peptide
  VARIANT 5: note = Xaa can be any naturally occurring amino acid
  VARIANT 11..13: note = Xaa can be any naturally occurring amino acid
  VARIANT 20: note = Xaa can be any naturally occurring amino acid
  VARIANT 29: note = Xaa can be any naturally occurring amino acid
  VARIANT 31: note = Xaa can be any naturally occurring amino acid
  VARIANT 33: note = Xaa can be any naturally occurring amino acid
  VARIANT 37..38: note = Xaa can be any naturally occurring amino acid
  VARIANT 40: note = Xaa can be any naturally occurring amino acid
  VARIANT 45: note = Xaa can be any naturally occurring amino acid
  VARIANT 48: note = Xaa can be any naturally occurring amino acid
  VARIANT 50: note = Xaa can be any naturally occurring amino acid
  VARIANT 55..57: note = Xaa can be any naturally occurring amino acid
  VARIANT 59: note = Xaa can be any naturally occurring amino acid
  VARIANT 61..62: note = Xaa can be any naturally occurring amino acid
  VARIANT 65..68: note = Xaa can be any naturally occurring amino acid
  VARIANT 70: note = Xaa can be any naturally occurring amino acid
  VARIANT 72: note = Xaa can be any naturally occurring amino acid
  VARIANT 74: note = Xaa can be any naturally occurring amino acid
  VARIANT 76: note = Xaa can be any naturally occurring amino acid
  VARIANT 79: note = Xaa can be any naturally occurring amino acid
  VARIANT 82: note = Xaa can be any naturally occurring amino acid
  VARIANT 84: note = Xaa can be any naturally occurring amino acid
  VARIANT 87: note = Xaa can be any naturally occurring amino acid
  VARIANT 91: note = Xaa can be any naturally occurring amino acid
  VARIANT 97: note = Xaa can be any naturally occurring amino acid
  VARIANT 101: note = Xaa can be any naturally occurring amino acid
  VARIANT 117: note = Xaa can be any naturally occurring amino acid
QVQLXQSGAEXXXPGASVKXSCKASGYTXTXYXMHWXXQXPGQGXEWXGXINPSXXXTXYXXKFXXXXTXTXDXSXSTXYMXLXSLXSEDXAVYYCXRGEXGGFAYWGQGTLVTVSX

SEQ ID NO: 437 - protein, 117 aa, synthetic construct
  REGION 1..117: note = Synthetic peptide
  VARIANT 20: note = Xaa can be any naturally occurring amino acid
  VARIANT 29: note = Xaa can be any naturally occurring amino acid
  VARIANT 31: note = Xaa can be any naturally occurring amino acid
  VARIANT 37: note = Xaa can be any naturally occurring amino acid
  VARIANT 45: note = Xaa can be any naturally occurring amino acid
  VARIANT 48: note = Xaa can be any naturally occurring amino acid
  VARIANT 56: note = Xaa can be any naturally occurring amino acid
  VARIANT 59: note = Xaa can be any naturally occurring amino acid
  VARIANT 61..62: note = Xaa can be any naturally occurring amino acid
  VARIANT 65..66: note = Xaa can be any naturally occurring amino acid
  VARIANT 68: note = Xaa can be any naturally occurring amino acid
  VARIANT 70: note = Xaa can be any naturally occurring amino acid
  VARIANT 74: note = Xaa can be any naturally occurring amino acid
  VARIANT 79: note = Xaa can be any naturally occurring amino acid
  VARIANT 84: note = Xaa can be any naturally occurring amino acid
  VARIANT 97: note = Xaa can be any naturally occurring amino acid
  VARIANT 101: note = Xaa can be any naturally occurring amino acid
QVQLVQSGAEVKKPGASVKXSCKASGYTXTXYTMHWXRQAPGQGXEWXGYINPSSXYTXYXXKFXXRXTXTADXSTSTXYMELXSLRSEDTAVYYCXRGEXGGFAYWGQGTLVTVSS

SEQ ID NO: 438 - protein, 112 aa, synthetic construct
  REGION 1..112: note = Synthetic peptide
  VARIANT 7: note = Xaa can be any naturally occurring amino acid
  VARIANT 14: note = Xaa can be any naturally occurring amino acid
  VARIANT 17..18: note = Xaa can be any naturally occurring amino acid
  VARIANT 31: note = Xaa can be any naturally occurring amino acid
  VARIANT 33: note = Xaa can be any naturally occurring amino acid
  VARIANT 39: note = Xaa can be any naturally occurring amino acid
  VARIANT 41..42: note = Xaa can be any naturally occurring amino acid
  VARIANT 44: note = Xaa can be any naturally occurring amino acid
  VARIANT 50..51: note = Xaa can be any naturally occurring amino acid
  VARIANT 55: note = Xaa can be any naturally occurring amino acid
  VARIANT 57: note = Xaa can be any naturally occurring amino acid
  VARIANT 81: note = Xaa can be any naturally occurring amino acid
  VARIANT 88: note = Xaa can be any naturally occurring amino acid
  VARIANT 92: note = Xaa can be any naturally occurring amino acid
  VARIANT 94..96: note = Xaa can be any naturally occurring amino acid
  VARIANT 99..100: note = Xaa can be any naturally occurring amino acid
  VARIANT 105: note = Xaa can be any naturally occurring amino acid
DVVMTQXPLSLPVXLGXXASISCRSSQSLVXSXGNTYLXWXXQXPGQSPXXNPSXTXTHYSGVPDRFSGSGSGTDFTLKIXRVEAEDXGVYXCXXXTHXXYTFGXGTKLEIK

SEQ ID NO: 439 - protein, 112 aa, synthetic construct
  REGION 1..112: note = Synthetic peptide
  VARIANT 33: note = Xaa can be any naturally occurring amino acid
  VARIANT 39: note = Xaa can be any naturally occurring amino acid
  VARIANT 55: note = Xaa can be any naturally occurring amino acid
  VARIANT 57: note = Xaa can be any naturally occurring amino acid
  VARIANT 81: note = Xaa can be any naturally occurring amino acid
  VARIANT 95..96: note = Xaa can be any naturally occurring amino acid
DVVMTQSPLSLPVTLGQPASISCRSSQSLVHSXGNTYLXWYQQRPGQSPRLLIYXVXNRFSGVPDRFSGSGSGTDFTLKIXRVEAEDVGVYYCSXXTHVPYTFGQGTKLEIK

SEQ ID NO: 440 - protein, 120 aa, synthetic construct
  REGION 1..120: note = Synthetic peptide
  VARIANT 5: note = Xaa can be any naturally occurring amino acid
  VARIANT 9: note = Xaa can be any naturally occurring amino acid
  VARIANT 11..12: note = Xaa can be any naturally occurring amino acid
  VARIANT 20: note = Xaa can be any naturally occurring amino acid
  VARIANT 38: note = Xaa can be any naturally occurring amino acid
  VARIANT 40..41: note = Xaa can be any naturally occurring amino acid
  VARIANT 43..44: note = Xaa can be any naturally occurring amino acid
  VARIANT 48: note = Xaa can be any naturally occurring amino acid
  VARIANT 61: note = Xaa can be any naturally occurring amino acid
  VARIANT 65: note = Xaa can be any naturally occurring amino acid
  VARIANT 67..68: note = Xaa can be any naturally occurring amino acid
  VARIANT 70: note = Xaa can be any naturally occurring amino acid
  VARIANT 72: note = Xaa can be any naturally occurring amino acid
  VARIANT 74: note = Xaa can be any naturally occurring amino acid
  VARIANT 76: note = Xaa can be any naturally occurring amino acid
  VARIANT 79: note = Xaa can be any naturally occurring amino acid
  VARIANT 82: note = Xaa can be any naturally occurring amino acid
  VARIANT 84: note = Xaa can be any naturally occurring amino acid
  VARIANT 87: note = Xaa can be any naturally occurring amino acid
  VARIANT 91: note = Xaa can be any naturally occurring amino acid
  VARIANT 116: note = Xaa can be any naturally occurring amino acid
QVQLXQSGXEXXKPGASVKXSCKASGYSFTGYNMNWVXQXXGXXLEWXGNIDPYYGGSTYXQKFXGXXTXTXDXSXSTXYMXLXSLXSEDXAVYYCARERSGYVFSAMDYWGQGTXVTVS

SEQ ID NO: 441 - protein, 120 aa, synthetic construct
  REGION 1..120: note = Synthetic peptide
  VARIANT 20: note = Xaa can be any naturally occurring amino acid
  VARIANT 48: note = Xaa can be any naturally occurring amino acid
  VARIANT 68: note = Xaa can be any naturally occurring amino acid
  VARIANT 70: note = Xaa can be any naturally occurring amino acid
  VARIANT 79: note = Xaa can be any naturally occurring amino acid
QVQLVQSGAEVKKPGASVKXSCKASGYSFTGYNMNWVRQAPGQGLEWXGNIDPYYGGSTYAQKFQGRXTXTRDTSTSTXYMELSSLRSEDTAVYYCARERSGYVFSAMDYWGQGTLVTVS

SEQ ID NO: 442 - protein, 112 aa, synthetic construct
  REGION 1..112: note = Synthetic peptide
  VARIANT 1: note = Xaa can be any naturally occurring amino acid
  VARIANT 3: note = Xaa can be any naturally occurring amino acid
  VARIANT 9: note = Xaa can be any naturally occurring amino acid
  VARIANT 15: note = Xaa can be any naturally occurring amino acid
  VARIANT 18..19: note = Xaa can be any naturally occurring amino acid
  VARIANT 21..22: note = Xaa can be any naturally occurring amino acid
  VARIANT 49: note = Xaa can be any naturally occurring amino acid
  VARIANT 51: note = Xaa can be any naturally occurring amino acid
  VARIANT 69: note = Xaa can be any naturally occurring amino acid
  VARIANT 78: note = Xaa can be any naturally occurring amino acid
  VARIANT 84: note = Xaa can be any naturally occurring amino acid
  VARIANT 93: note = Xaa can be any naturally occurring amino acid
  VARIANT 105: note = Xaa can be any naturally occurring amino acid
  VARIANT 111: note = Xaa can be any naturally occurring amino acid
XIXMTQSPXSLAVSXGEXXTXXCKSSQSVLFSSNQKNYLAWYQQKPGQXPXLLIYWASTRESGVPDRFXGSGSGTDFXLTISSXQAEDVAVYXCHQYLSSRTFGXGTKLEXK

SEQ ID NO: 443 - protein, 112 aa, synthetic construct
  REGION 1..112: note = Synthetic peptide
  VARIANT 19: note = Xaa can be any naturally occurring amino acid
  VARIANT 21: note = Xaa can be any naturally occurring amino acid
  VARIANT 84: note = Xaa can be any naturally occurring amino acid
DIVMTQSPDSLAVSLGERXTXNCKSSQSVLFSSNQKNYLAWYQQKPGQPPKLLIYWASTRESGVPDRFSGSGSGTDFTLTISSXQAEDVAVYYCHQYLSSRTFGQGTKLEIK

SEQ ID NO: 444 - protein, 117 aa, synthetic construct
  REGION 1..117: note = Synthetic peptide
  VARIANT 1: note = Xaa can be any naturally occurring amino acid
  VARIANT 5: note = Xaa can be any naturally occurring amino acid
  VARIANT 9: note = Xaa can be any naturally occurring amino acid
  VARIANT 11..12: note = Xaa can be any naturally occurring amino acid
  VARIANT 20: note = Xaa can be any naturally occurring amino acid
  VARIANT 38: note = Xaa can be any naturally occurring amino acid
  VARIANT 40..41: note = Xaa can be any naturally occurring amino acid
  VARIANT 43..44: note = Xaa can be any naturally occurring amino acid
  VARIANT 48: note = Xaa can be any naturally occurring amino acid
  VARIANT 61: note = Xaa can be any naturally occurring amino acid
  VARIANT 63: note = Xaa can be any naturally occurring amino acid
  VARIANT 65: note = Xaa can be any naturally occurring amino acid
  VARIANT 67: note = Xaa can be any naturally occurring amino acid
  VARIANT 69..70: note = Xaa can be any naturally occurring amino acid
  VARIANT 72..74: note = Xaa can be any naturally occurring amino acid
  VARIANT 76: note = Xaa can be any naturally occurring amino acid
  VARIANT 79: note = Xaa can be any naturally occurring amino acid
  VARIANT 84: note = Xaa can be any naturally occurring amino acid
  VARIANT 87: note = Xaa can be any naturally occurring amino acid
  VARIANT 91: note = Xaa can be any naturally occurring amino acid
  VARIANT 93: note = Xaa can be any naturally occurring amino acid
  VARIANT 112..113: note = Xaa can be any naturally occurring amino acid
XVQLXQSGXEXXKPGASVKXSCKASGYRFTDYNMHWVXQXXGXXLEWXGYINPNNGGTNYXQXFXGXVXXTXXXSXSTXYMELXSLXSEDXAXYYCARDYLYFFDCWGQGTXXTVSS

SEQ ID NO: 445 - protein, 107 aa, synthetic construct
  REGION 1..107: note = Synthetic peptide
  VARIANT 9: note = Xaa can be any naturally occurring amino acid
  VARIANT 11: note = Xaa can be any naturally occurring amino acid
  VARIANT 15: note = Xaa can be any naturally occurring amino acid
  VARIANT 17..18: note = Xaa can be any naturally occurring amino acid
  VARIANT 43: note = Xaa can be any naturally occurring amino acid
  VARIANT 45: note = Xaa can be any naturally occurring amino acid
  VARIANT 70: note = Xaa can be any naturally occurring amino acid
  VARIANT 72..74: note = Xaa can be any naturally occurring amino acid
  VARIANT 80: note = Xaa can be any naturally occurring amino acid
  VARIANT 84..85: note = Xaa can be any naturally occurring amino acid
  VARIANT 100: note = Xaa can be any naturally occurring amino acid
DIQMTQSPXSXSASXGXXVTITCLASQTIGTWLAWYQQKPGKXPXLLIYAAASLADGVPSRFSGSGSGTXFXXXISSLQXEDFXXYYCQQLYSIPRTFGXGTKLEIK

SEQ ID NO: 446 - protein, 107 aa, synthetic construct
  REGION 1..107: note = Synthetic peptide
  VARIANT 1: note = Xaa can be any naturally occurring amino acid
  VARIANT 15: note = Xaa can be any naturally occurring amino acid
  VARIANT 18..19: note = Xaa can be any naturally occurring amino acid
  VARIANT 42: note = Xaa can be any naturally occurring amino acid
  VARIANT 49: note = Xaa can be any naturally occurring amino acid
  VARIANT 63: note = Xaa can be any naturally occurring amino acid
  VARIANT 75..76: note = Xaa can be any naturally occurring amino acid
  VARIANT 78: note = Xaa can be any naturally occurring amino acid
  VARIANT 80: note = Xaa can be any naturally occurring amino acid
  VARIANT 84: note = Xaa can be any naturally occurring amino acid
  VARIANT 88: note = Xaa can be any naturally occurring amino acid
  VARIANT 93: note = Xaa can be any naturally occurring amino acid
XVQLVESGGGLVQPXGSXXLSCAASGFTFSSFGMHWVRQAPXKGLEWVXYISSDSRTIYYADXVKGRFTISRDNXXNXLXLQMXSLRXEDTAXYYCARDYGRTYEAY

SEQ ID NO: 447 - protein, 111 aa, synthetic construct
  REGION 1..111: note = Synthetic peptide
  VARIANT 4: note = Xaa can be any naturally occurring amino acid
  VARIANT 9: note = Xaa can be any naturally occurring amino acid
  VARIANT 17: note = Xaa can be any naturally occurring amino acid
  VARIANT 22: note = Xaa can be any naturally occurring amino acid
  VARIANT 64: note = Xaa can be any naturally occurring amino acid
  VARIANT 78: note = Xaa can be any naturally occurring amino acid
  VARIANT 80..84: note = Xaa can be any naturally occurring amino acid
  VARIANT 87: note = Xaa can be any naturally occurring amino acid
  VARIANT 89: note = Xaa can be any naturally occurring amino acid
  VARIANT 104: note = Xaa can be any naturally occurring amino acid
  VARIANT 110: note = Xaa can be any naturally occurring amino acid
DIVXTQSPXSLAVSLGXRATIXCRASKSVSTSGYSYIHWYQQKPGQPPKLLIYLASNLESGVPXRFSGSGSGTDFTLXIXXXXXEDXAXYYCQHSRELPLTFGXGTKLEXK

SEQ ID NO: 448 - protein, 111 aa, synthetic construct
  REGION 1..111: note = Synthetic peptide
  VARIANT 4: note = Xaa can be any naturally occurring amino acid
  VARIANT 82: note = Xaa can be any naturally occurring amino acid
  VARIANT 110: note = Xaa can be any naturally occurring amino acid
DIVXTQSPDSLAVSLGERATINCRASKSVSTSGYSYIHWYQQKPGQPPKLLIYLASNLESGVPDRFSGSGSGTDFTLTISSXQAEDVAVYYCQHSRELPLTFGQGTKLEXK

SEQ ID NO: 449 - protein, 7 aa, synthetic construct
  REGION 1..7: note = Synthetic peptide
  VARIANT 6: note = Xaa is T, V, F, or D
SSVSSXY

SEQ ID NO: 450 - skipped

SEQ ID NO: 451 - protein, 9 aa, synthetic construct
  REGION 1..9: note = Synthetic peptide
  VARIANT 2: note = Xaa is Q, H or S
  VARIANT 4: note = Xaa is H, Y, Q, or S
HXYXRSPLT

SEQ ID NO: 452 - protein, 7 aa, synthetic construct
  REGION 1..7: note = Synthetic peptide
  VARIANT 5: note = Xaa is T, V, D, or S
YTFTXYT

SEQ ID NO: 453 - protein, 9 aa, synthetic construct
  REGION 1..9: note = Synthetic peptide
  VARIANT 2: note = Xaa is N, Q, H, D, S, R, or A
AXGDYYVAY

SEQ ID NO: 454 - protein, 9 aa, synthetic construct
  REGION 1..9: note = Synthetic peptide
  VARIANT 2: note = Xaa is H, Q, S, or T
  VARIANT 5: note = Xaa is T, S, N, or G
QXHYXVPWT

SEQ ID NO: 455 - protein, 7 aa, synthetic construct
  REGION 1..7: note = Synthetic peptide
  VARIANT 5: note = Xaa is N, S, R, q, s, or a
  VARIANT 7: note = Xaa is w, h, y, or f
FTFSXYX

SEQ ID NO: 456 - protein, 10 aa, synthetic construct
  REGION 1..10: note = Synthetic peptide
  VARIANT 5: note = Xaa is S, N, A, or T
  VARIANT 7: note = Xaa is Q, S,A, or N
IRLKXDXYAT

SEQ ID NO: 457 - protein, 8 aa, synthetic construct
  REGION 1..8: note = Synthetic peptide
  VARIANT 1: note = Xaa is N, D, A, or T
  VARIANT 8: note = Xaa is S, T, A, C, Y
XDGPPSGX

SEQ ID NO: 458 - protein, 11 aa, synthetic construct
  REGION 1..11: note = Synthetic peptide
  VARIANT 7: note = Xaa is D, N, E, Q, S, or A
  VARIANT 9: note = Xaa is Q, S, A, D, or N
QSLVHSXGXTY

SEQ ID NO: 459 - skipped

SEQ ID NO: 460 - protein, 9 aa, synthetic construct
  REGION 1..9: note = Synthetic peptide
  VARIANT 2: note = Xaa is Q, H, or T
  VARIANT 3: note = Xaa is S, G, T, or D
SXXTHVPYT

SEQ ID NO: 461 - protein, 9 aa, synthetic construct
  REGION 1..9: note = Synthetic peptide
  VARIANT 3: note = Xaa is F, Y, S, or T
  VARIANT 5: note = Xaa is S, T, Y , or D
YTXTXYTMH

SEQ ID NO: 462 - protein, 8 aa, synthetic construct
  REGION 1..8: note = Synthetic peptide
  VARIANT 2: note = Xaa is Q, S, A, or N
  VARIANT 6: note = Xaa is T, S, V, D, or G
IXPSSXYT

SEQ ID NO: 463 - protein, 10 aa, synthetic construct
  REGION 1..10: note = Synthetic peptide
  VARIANT 1: note = Xaa is S, A, T, or V
  VARIANT 5: note = Xaa is L, V, or F
XRGEXGGFAY

SEQ ID NO: 464 - protein, 6 aa, synthetic construct
  REGION 1..6: note = Synthetic peptide
  VARIANT 6: note = Xaa is W, H, Y, or F
QTIGYX

SEQ ID NO: 465 - protein, 8 aa, synthetic construct
  REGION 1..8: note = Synthetic peptide
  VARIANT 3: note = Xaa is R or T
  VARIANT 8: note = Xaa is N, Q, S, or A
GYXFTDYX

SEQ ID NO: 466 - protein, 8 aa, synthetic construct
  REGION 1..8: note = Synthetic peptide
  VARIANT 2: note = Xaa is N, Q, S, or A
  VARIANT 4: note = Xaa is N, Q, S, or A
  VARIANT 5: note = Xaa is N, Q, S, or A
IXPXXGGT

SEQ ID NO: 467 - protein, 8 aa, synthetic construct
  REGION 1..8: note = Synthetic peptide
  VARIANT 8: note = Xaa is C, Y, S, or A
DYLYFFDX

SEQ ID NO: 468 - protein, 8 aa, synthetic construct
  REGION 1..8: note = Synthetic peptide
  VARIANT 4: note = Xaa is D, E, S, or A
ISSXSRTI

SEQ ID NO: 469 - protein, 9 aa, synthetic construct
  REGION 1..9: note = Synthetic peptide
DYGRTYEAY

SEQ ID NO: 470 - protein, 12 aa, synthetic construct
  REGION 1..12: note = Synthetic peptide
  VARIANT 8: note = Xaa is Q, S, A, D, or N
  VARIANT 11: note = Xaa is Q, S, A, D, or N
QSVLFSSXQKXY

SEQ ID NO: 471 - skipped

SEQ ID NO: 472 - protein, 8 aa, synthetic construct
  REGION 1..8: note = Synthetic peptide
  VARIANT 8: note = Xaa is N, Q, S, or A
GYSFTFYX

SEQ ID NO: 473 - protein, 8 aa, synthetic construct
  REGION 1..8: note = Synthetic peptide
  VARIANT 2: note = Xaa is A, S, E, or D
IXPYYGGS

SEQ ID NO: 474 - protein, 12 aa, synthetic construct
  REGION 1..12: note = Synthetic peptide
ERSGYVFSAMDY

SEQ ID NO: 475 - protein, 8 aa, synthetic construct
  REGION 1..8: note = Synthetic peptide
  VARIANT 2: note = Xaa is Q, S, A, or N
IXPSSGYT

SEQ ID NO: 476 - protein, 6 aa, synthetic construct
  REGION 1..6: note = Synthetic peptide
  VARIANT 2: note = Xaa is Q, S, A, D, or N
EXIYSY

SEQ ID NO: 477 - skipped

SEQ ID NO: 478 - protein, 116 aa, synthetic construct
  REGION 1..116: note = Synthetic peptide
  VARIANT 20: note = Xaa is M or V
  VARIANT 31: note = Xaa is T, V, D, or S
  VARIANT 48: note = Xaa is I or M
  VARIANT 52: note = Xaa is Q, S, A, or N
  VARIANT 70: note = Xaa is L or M
  VARIANT 74: note = Xaa is T or K
  VARIANT 98: note = Xaa is N, Q, H, D, S, R,or A
QVQLVQSGAEVKKPGASVKXSCKASGYTFTXYTMHWVRQAPGQGLEWXGFIXPSSGYTDYAQKFQGRVTXTADXSTSTVYMELSSLRSEDTAVYYCAXGDYYVAYWGQGTLVTVSS

SEQ ID NO: 479 - protein, 108 aa, synthetic construct
  REGION 1..108: note = Synthetic peptide
  VARIANT 4: note = Xaa is L or M
  VARIANT 21: note = Xaa is M or I
  VARIANT 32: note = Xaa is T, V, F, or D
  VARIANT 48: note = Xaa is W or L
  VARIANT 51: note = Xaa is S, t, Q or A
  VARIANT 53: note = Xaa is S,T, D or Q
  VARIANT 79: note = Xaa is M or L
  VARIANT 84: note = Xaa is A or F
  VARIANT 91: note = Xaa is Q, H or S
  VARIANT 93: note = Xaa is H, Y, Q, or S
DIQXTQSPSSLSASVGDRVTXTCTASSSVSSXYFHWYQQKPGKAPKLXIYXTXNLASGVPSRFSGSGSGTDYTLTISSXQPEDXATYYCHXYXRSPLTFGQGTKLEIK

SEQ ID NO: 480 - protein, 117 aa, synthetic construct
  REGION 1..117: note = Synthetic peptide
  VARIANT 31: note = Xaa is N, S, R, Q or A
  VARIANT 33: note = Xaa is W, H, Y or F
  VARIANT 55: note = Xaa is S, N, A, or T
  VARIANT 57: note = Xaa is Q, S, A, or N
  VARIANT 99: note = Xaa is N, D, or T
  VARIANT 106: note = Xaa is S, T, A, C, or Y
EVQLLESGGGLVQPGGSMRLSCAASGFTFSXYXMNWVRQAPGKGLEWVAQIRLKXDXYATHYADSVKGRFTISRDDSKNTVYLQMNSLRAEDTGVYYCXDGPPSGXWGQGTLLTVSS

SEQ ID NO: 481 - protein, 107 aa, synthetic construct
  REGION 1..107: note = Synthetic peptide
  VARIANT 28: note = Xaa is Q, S, A, D, or N
  VARIANT 48: note = Xaa is V or I
  VARIANT 50: note = Xaa is S, T, Q or A
  VARIANT 84: note = Xaa is G or A
  VARIANT 90: note = Xaa is H, Q, S or T
  VARIANT 93: note = Xaa is T, S, N, or G
DIQMTQSPSSLSASVGDRVTITCRISEXIYSYLAWYQQKPGKAPKLLXYXAKILVEGVPSRFSGSGSGTDFTLTISSLQPEDFXTYYCQXHYXVPWTFGQGTKLEIK

SEQ ID NO: 482 - protein, 117 aa, synthetic construct
  REGION 1..117: note = Synthetic peptide
  VARIANT 20: note = Xaa is M or V
  VARIANT 29: note = Xaa is F, Y, S or T
  VARIANT 31: note = Xaa is S, T, Y, or D
  VARIANT 37: note = Xaa is I or V
  VARIANT 45: note = Xaa is Q or L
  VARIANT 48: note = Xaa is I or M
  VARIANT 52: note = Xaa is Q, S, A, or N
  VARIANT 56: note = Xaa is T, S, V, D or G
  VARIANT 61: note = Xaa is I or A
  VARIANT 62: note = Xaa is K or Q
  VARIANT 65: note = Xaa is K or Q
  VARIANT 66: note = Xaa is D or G
  VARIANT 68: note = Xaa is A or V
  VARIANT 70: note = Xaa is L or M
  VARIANT 74: note = Xaa is T or K
  VARIANT 79: note = Xaa is A or V
  VARIANT 97: note = Xaa is S, A, T, or V
  VARIANT 101: note = Xaa is L, V, or F
  VARIANT 101: note = Xaa can be any naturally occurring amino acid
QVQLVQSGAEVKKPGASVKXSCKASGYTXTXYTMHWXRQAPGQGXEWXGYIXPSSXYTHYXXKFXXRXTXTADXSTSTXYMELSSLRSEDTAVYYCXRGEXGGFAYWGQGTLVTVSS

SEQ ID NO: 483 - protein, 112 aa, synthetic construct
  REGION 1..112: note = Synthetic peptide
  VARIANT 33: note = Xaa is D, N, E, Q, S, or A
  VARIANT 35: note = Xaa is Q, S, A, D, or N
  VARIANT 55: note = Xaa is K, Q, or R
  VARIANT 57: note = Xaa is S, T, or V
  VARIANT 95: note = Xaa is Q, H, or T
  VARIANT 96: note = Xaa is S, G, T, or D
DVVMTQSPLSLPVTLGQPASISCRSSQSLVHSDGXTYLNWYQQRPGQSPRLLIYXVXNRFSGVPDRFSGSGSGTDFTLKISRVEAEDVGVYYCSXXTHVPYTFGQGTKLEIK

SEQ ID NO: 484 - protein, 121 aa, synthetic construct
  REGION 1..121: note = Synthetic peptide
  VARIANT 20: note = Xaa is I or V
  VARIANT 33: note = Xaa is N, Q, S, or A
  VARIANT 48: note = Xaa is I or M
  VARIANT 52: note = Xaa is A, S, E or D
  VARIANT 68: note = Xaa is A or V
  VARIANT 70: note = Xaa is L or M
  VARIANT 79: note = Xaa is A or V
QVQLVQSGAEVKKPGASVKXSCKASGYSFTGYXMNWVRQAPGQGLEWXGNIXPYYGGSTYAQKFQGRXTXTVDTSTSTXYMELSSLRSEDTAVYYCARERSGYVFSAMDYWGQGTLVTVSS

SEQ ID NO: 485 - protein, 112 aa, synthetic construct
  REGION 1..112: note = Synthetic peptide
  VARIANT 19: note = Xaa is V or A
  VARIANT 21: note = Xaa is M or I
  VARIANT 34: note = Xaa is Q, S, A, D, or N
  VARIANT 37: note = Xaa is Q, S, A, D, or N
  VARIANT 56: note = Xaa is H, Y, F, or W
  VARIANT 84: note = Xaa is V or L
DIVMTQSPDSLAVSLGERXTXNCKSSQSVLFSSXQKXYLAWYQQKPGQPPKLLIYXASTRESGVPDRFSGSGSGTDFTLTISSXQAEDVAVYYCHQYLSSRTFGQGTKLEIK

SEQ ID NO: 486 - protein, 118 aa, synthetic construct
  REGION 1..118: note = Synthetic peptide
  VARIANT 54: note = Xaa is D, E, S, or A
EVQLVESGGGLVQPGGSLRLSCAASGFTFSSFGMHWVRQAPGKGLEWVAYISSXSRTIYYADSVKGRFTISRDNAKNSLYLQMNSLRAEDTAVYYCARDYGRTYEAYWGQGTLVTVSS

SEQ ID NO: 487 - protein, 111 aa, synthetic construct
  REGION 1..111: note = Synthetic peptide
  VARIANT 4: note = Xaa is M or L
  VARIANT 82: note = Xaa is V or L
  VARIANT 110: note = Xaa is I or L
DIVXTQSPDSLAVSLGERATINCRASKSVSTSGYSYIHWYQQKPGQPPKLLIYLASNLESGVPDRFSGSGSGTDFTLTISSXQAEDVAVYYCQHSRELPLTFGQGTKLEIK

SEQ ID NO: 488 - protein, 117 aa, synthetic construct
  REGION 1..117: note = Synthetic peptide
  VARIANT 28: note = Xaa is R or T
  VARIANT 33: note = Xaa is N, Q, S or A
  VARIANT 52: note = Xaa is N, Q, S or A
  VARIANT 54: note = Xaa is N, Q, S or A
  VARIANT 55: note = Xaa is N, Q, S, or A
  VARIANT 106: note = Xaa is C, Y, S, or A
QVQLVQSGAEVKKPGASVKMSCKASGYXFTDYXMHWVRQAPGQGLEWIGYIXPXXGGTNYAQKFQGRATLTVDTSTSTAYMELSSLRSEDTAVYYCARDYLYFFDXWGQGTLLTVSS

SEQ ID NO: 489 - protein, 107 aa, synthetic construct
  REGION 1..107: note = Synthetic peptide
  VARIANT 24: note = Xaa is L or R
  VARIANT 32: note = Xaa is W, H, Y, or F
DIQMTQSPSSLSASVGDRVTITCLASQTIGTXLAWYQQKPGKAPKLLIYAAASLADGVPSRFSGSGSGTDFTFTISSLQPEDFVTYYCQQLYSIPRTFGQGTKLEIK

SEQ ID NO: 490 - protein, 117 aa, synthetic construct
  REGION 1..117: note = Synthetic Polypeptide
EVQLLESGGGLVQPGGSMRLSCAASGFTFSNYWMNWVRQAPGKGLEWIAQIRLKSDNYATHYTDSVKGRFTISRDDSKRTVYLQMNSLRAEDTGTYYCSDGPPSGSWGQGTLLTVSS

SEQ ID NO: 491 - protein, 117 aa, synthetic construct
  REGION 1..117: note = Synthetic Polypeptide
EVQLLESGGGLVQPGGSMRLSCAASGFTFSNYWMNWVRQAPGKGLEWIAQIRLKSDNYATHYADSVKGRFTISRDDSKRTVYLQMNSLRAEDTGTYYCSDGPPSGSWGQGTLLTVSS

SEQ ID NO: 492 - protein, 117 aa, synthetic construct
  REGION 1..117: note = Synthetic Polypeptide
EVQLLESGGGLVQPGGSMRLSCAASGFTFSNYWMNWVRQAPGKGLEWIAQIRLKSDNYVTHYTDSVKGRFTISRDDSKRTVYLQMNSLRAEDTGIYYCSDGPPSGSWGQGTLLTVSS

SEQ ID NO: 493 - protein, 117 aa, synthetic construct
  REGION 1..117: note = Synthetic Polypeptide
EVQLLESGGGLVQPGGSMRLSCAASGFTFSNYWMNWVRQAPGKGLEWIAQIRLKSDNYATHYTDSVKGRFTISRDDSKSTVYLQMNSLRAEDTGTYYCNDGPPSGSWGQGTLLTVSS

SEQ ID NO: 494 - protein, 117 aa, synthetic construct
  REGION 1..117: note = Synthetic Polypeptide
EVQLLESGGGLVQPGGSMRLSCAASGFTFSNYWMNWVRQAPGKGLEWLAQIRLKSDNYATHYTDSVKGRFTISRDDSKRTVYLQMNSLRAEDTGIYYCSDGPPSGSWGQGTLLTVSS

SEQ ID NO: 495 - protein, 117 aa, synthetic construct
  REGION 1..117: note = Synthetic Polypeptide
EVQLLESGGGLVQPGGSMRLSCAASGFTFSNYWMNWVRQAPGKGLEWLAQIRLKSDNYVTHYADSVKGRFTISRDDSKRTVYLQMNSLRAEDTGTYYCNDGPPSGSWGQGTLLTVSS

SEQ ID NO: 496 - protein, 116 aa, synthetic construct
  REGION 1..116: note = Synthetic Polypeptide
QVQLVQSGAEVKKPGASVKMSCKASGYTFTTYTIHWVRQAPGQGLEWIGFINPSSGYTEYAQKFQGRVTLTADKSTSTVYMELSSLRSEDTAVYFCANGDYYVAYWGQGTLVTVSS

SEQ ID NO: 497 - protein, 116 aa, synthetic construct
  REGION 1..116: note = Synthetic Polypeptide
QVQLVQSGAEVKKPGASVKMSCKASGYTFTTYTMHWVRQAPGQGLEWIGVINPSSGYTEYAQKFQGRVTLTADKSTSTVYMELSSLRSEDTAVYFCANGDYYVGYWGQGTLVTVSS

SEQ ID NO: 498 - protein, 116 aa, synthetic construct
  REGION 1..116: note = Synthetic Polypeptide
QVQLVQSGAEVKKPGASVKMSCKASGYTFTTYTIHWVRQAPGQGLEWIGVINPSSGYTDYAQKFQGRVTLTADKSTSTVYMELSSLRSEDTAVYFCANGDYYVGYWGQGTLVTVSS

SEQ ID NO: 499 - protein, 116 aa, synthetic construct
  REGION 1..116: note = Synthetic Polypeptide
QVQLVQSGAEVKKPGASVKMSCKASGYTFTTYTMHWVRQAPGQGLEWIGFINPSSGYTEYAQKFQGRVTLTADKSTSTVYMELSSLRSEDTAVYYCANGDYYVGYWGQGTLVTVSS

SEQ ID NO: 500 - protein, 116 aa, synthetic construct
  REGION 1..116: note = Synthetic Polypeptide
QVQLVQSGAEVKKPGASVKMSCKASGYTFTTYTIHWVRQAPGQGLEWIGVINPSSGYTEYAQKFQGRVTLTADKSTSTVYMELSSLRSEDTAVYFCANGDYYVAYWGQGTLVTVSS

SEQ ID NO: 501 - protein, 116 aa, synthetic construct
  REGION 1..116: note = Synthetic Polypeptide
QVQLVQSGAEVKKPGASVKMSCKASGYTFTTYTMHWVRQAPGQGLEWIGFINPSSGYTEYAQKFQGRVTLTADKSTSTVYMELSSLRSEDTAVYFCANGDYYVGYWGQGTLVTVSS

SEQ ID NO: 502 - protein, 117 aa, synthetic construct
  REGION 1..117: note = Synthetic Polypeptide
  VARIANT 48: note = Xaa is any aliphatic amino acid, optionally Ile or Leu
  VARIANT 59: note = Xaa is any aliphatic amino acid, optionally, Ala or Val
  VARIANT 63: note = Xaa is any aliphatic or any amino acid with a polar side chain, optionally, Ala or Thr
  VARIANT 79: note = Xaa is any basic amino acid or any amino acid with a polar side chain, optionally Arg or Ser
  VARIANT 95: note = Xaa is any aliphatic amino acid or any amino acid with a polar side chain, optionally, Thr or Ile
  VARIANT 99: note = Xaa is any acidic amino acid or any amino acid with a polar side chain, optionally, Ser or Asn
EVQLLESGGGLVQPGGSMRLSCAASGFTFSNYWMNWVRQAPGKGLEWXAQIRLKSDNYXTHYXDSVKGRFTISRDDSKXTVYLQMNSLRAEDTGXYYCXDGPPSGSWGQGTLLTVSS

SEQ ID NO: 503 - protein, 116 aa, synthetic construct
  REGION 1..116: note = Synthetic Polypeptide
  VARIANT 34: note = Xaa is any aliphatic amino acid or any amino acid comprising a sulfur containing side chain; optionally, Ile or Met
  VARIANT 50: note = Xaa is any aliphatic amino acid or any aromatic amino acid, optionally, Phe or Val
  VARIANT 59: note = Xaa is any acidic amino acid, optionally, Glu or Asp
  VARIANT 95: note = Xaa is any aromatic amino acid, optionally, Phe or Tyr
  VARIANT 104: note = Xaa is any aliphatic amino acid, optionally, Gly or Ala
QVQLVQSGAEVKKPGASVKMSCKASGYTFTTYTXHWVRQAPGQGLEWIGXINPSSGYTXYAQKFQGRVTLTADKSTSTVYMELSSLRSEDTAVYXCANGDYYVXYWGQGTLVTVSS

SEQ ID NO: 504 - protein, 8 aa, synthetic construct
  REGION 1..8: note = Synthetic Polypeptide
GYTFTTYT

SEQ ID NO: 505 - protein, 8 aa, synthetic construct
  REGION 1..8: note = Synthetic Polypeptide
INPSSGYT

SEQ ID NO: 506 - protein, 9 aa, synthetic construct
  REGION 1..9: note = Synthetic Polypeptide
  VARIANT 8: note = Xaa is any aliphatic amino acid, optionally, Gly or Ala
ANGDYYVXY

SEQ ID NO: 507 - protein, 8 aa, synthetic construct
  REGION 1..8: note = Synthetic Polypeptide
GFTFSNYW

SEQ ID NO: 508 - protein, 10 aa, synthetic construct
  REGION 1..10: note = Synthetic Polypeptide
  VARIANT 9: note = Xaa is any aliphatic amino acid, optionally, Ala or Val
IRLKSDNYXT

SEQ ID NO: 509 - protein, 8 aa, synthetic construct
  REGION 1..8: note = Synthetic Polypeptide
  VARIANT 1: note = Xaa is any acidic amino acid or any amino acid with a polar side chain, optionally, Ser or Asn
XDGPPSGS

SEQ ID NO: 510 - protein, 117 aa, synthetic construct
  REGION 1..117: note = Synthetic Polypeptide
EVKLEESGGGLVQPGGSMKLSCVASGFTFSNYWMNWVRQSPEKGLEWVAQIRLKSDNYATHYAESVKGRFTISRDDSKSSVYLQMNNLRAEDTGIYYCNDGPPSGCWGQGTTLTVSS

SEQ ID NO: 511 - protein, 107 aa, synthetic construct
  REGION 1..107: note = Synthetic Polypeptide
DIQMTQSPASLSASVGETVTITCRASENIYSYLAWYQQKQGKSPQLLVYNAKILVEGVPSRFSGSGSGTQFSLKINSLQPEDFGNYYCQHHYTVPWTFGGGTKLEIK

SEQ ID NO: 512 - protein, 108 aa, synthetic construct
  REGION 1..108: note = Synthetic Polypeptide
QIVLTQSPAIMSASLGERVTMTCTASSSVSSSYLHWYQQKPGSSPKLWIYSTSNLASGVPARFSGSGSGTSYSLTISSMEAEDAATYYCHQYHRSPLTFGAGTKLELK

SEQ ID NO: 513 - protein, 116 aa, synthetic construct
  REGION 1..116: note = Synthetic Polypeptide
QVQLQQSAAELARPGASVKMSCKASGYTFTSYTMHWVKQRPGQGLEWIGFINPSSGYTDYNQKFKDKTTLTADKSSSTAYMQLSSLTSEDSAVYYCANGDYYVAYWGQGTLVTVSA